European Patent Specification EP 3 555 298 B1, published April 17, 2024. Title: POLYNUCLEOTIDE SHUFFLING METHOD. Applicant: Universiteit Antwerpen Universiteit Gent. The sequence listing filed with the application follows.

SEQUENCE LISTING (21 sequences)

SEQ ID NO: 1 - DNA, 20 bp, Artificial Sequence
  pVTSE1 Forward Primer
ggtgctgagacctctagagg

SEQ ID NO: 2 - DNA, 20 bp, Artificial Sequence
  pVTSE1 Reverse Primer
catggtgagaccaagcttgg

SEQ ID NO: 3 - DNA, 20 bp, Artificial Sequence
  pVTSE2 Forward Primer
gcaggtgagacctctagagg

SEQ ID NO: 4 - DNA, 20 bp, Artificial Sequence
  pVTSE2 Reverse Primer
tgcactgagaccaagcttgg

SEQ ID NO: 5 - DNA, 20 bp, Artificial Sequence
  pVTSE3 Forward Primer
ggaagcgagacctctagagg

SEQ ID NO: 6 - DNA, 20 bp, Artificial Sequence
  pVTSE3 Reverse Primer
acctgtgagaccaagcttgg

SEQ ID NO: 7 - DNA, 20 bp, Artificial Sequence
  pVTSE4 Forward Primer
aagtaggagacctctagagg

SEQ ID NO: 8 - DNA, 20 bp, Artificial Sequence
  pVTSE4 Reverse Primer
gcttctgagaccaagcttgg

SEQ ID NO: 9 - DNA, 3811 bp, Artificial Sequence
  pVTSEII Vector
agcttgacgtcaggtggcacttttcggggaaatgtgcgcggaacccctatttgtttatttttctaaatacattcaaatatgtatccgctcatgagacaataaccctgataaatgcttcaataatattgaaaaaggaagagtatgagtattcaacatttccgtgtcgcccttattcccttttttgcggcattttgccttcctgtttttgctcacccagaaacgctggtgaaagtaaaagatgctgaagatcagttgggtgcacgagtgggttacatcgaactggatctcaacagcggtaagatccttgagagttttcgccccgaagaacgttttccaatgatgagcacttttaaagttctgctatgtggcgcggtattatcccgtattgacgccgggcaagagcaactcggtcgccgcatacactattctcagaatgacttggttgagtactcaccagtcacagaaaagcatcttacggatggcatgacagtaagagaattatgcagtgctgccataaccatgagtgataacactgcggccaacttacttctgacaacgatcggaggaccgaaggagctaaccgcttttttgcacaacatgggggatcatgtaactcgccttgatcgttgggaaccggagctgaatgaagccataccaaacgacgagcgtgacaccacgatgcctgtagcaatggcaacaacgttgcgcaaactattaactggcgaactacttactctagcttcccggcaacaattaatagactggatggaggcggataaagttgcaggaccacttctgcgctcggcccttccggctggctggtttattgctgataaatctggagccggtgagcgtggttctcgcggtatcattgcagcactggggccagatggtaagccctcccgtatcgtagttatctacacgacggggagtcaggcaactatggatgaacgaaatagacagatcgctgagataggtgcctcactgattaagcattggtaactgtcagaccaagtttactcatatatactttagattgatttaaaacttcatttttaatttaaaaggatctaggtgaagatcctttttgataatctcatgaccaaaatcccttaacgtgagttttcgttccactgagcgtcagaccccgtagaaaagatcaaaggatcttcttgagatcctttttttctgcgcgtaatctgctgcttgcaaacaaaaaaaccaccgctaccagcggtggtttgtttgccggatcaagagctaccaactctttttccgaaggtaactggcttcagcagagcgcagataccaaatactgttcttctagtgtagccgtagttaggccaccacttcaagaactctgtagcaccgcctacatacctcgctctgctaatcctgttaccagtggctgctgccagtggcgataagtcgtgtcttaccgggttggactcaagacgatagttaccggataaggcgcagcggtcgggctgaacggggggttcgtgcacacagcccagcttggagcgaacgacctacaccgaactgagatacctacagcgtgagctatgagaaagcgccacgcttcccgaagggagaaaggcggacaggtatccggtaagcggcagggtcggaacaggagagcgcacgagggagcttccagggggaaacgcctggtatctttatagtcctgtcgggtttcgccacctctgacttgagcgtcgatttttgtgatgctcgtcaggggggcggagcctatggaaaaacgccagcaacgcggcctttttacggttcctggccttttgctggccttttgctcacatgttctttcctgcgttatcccctgattctgtggataaccgtattaccgcctttgagtgtctagatagtcttcgacgtccacatatacctgccgttcactattatttagtgaaatgagatattatgatattttctgaattgtgattaaaaaggcaactttatgcccatgcaacagaaactataaaaaatacagagaatgaaaagaaacagatagattttttagttctttaggcccgtagtctgcaaatccttttatgattttctatcaaacaaaagaggaaaatagaccagttgcaatccaaacgagagtctaatagaatgaggtcgaaaagtaaatcgcgcgggtttgttactgataaagcaggcaagacctaaaatgtgtaaagggcaaagtgtatactttggcgtcaccccttacatattttaggtctttttttattgtgcgtaactaacttgccatcttcaaacaggagggctggaagaagcagaccgctaacacagtacataaaaaaggagacatgaacgatgaacatcaaaaagtttgcaaaacaagcaacagtattaacctttactaccgcactgctggcaggaggcgcaactcaagcgtttgcgaaagaaacgaaccaaaagccatataaggaaacatacggcatttcccatattacacgccatgatatgctgcaaatccctgaacagcaaaaaaatgaaaaatataaagttcctgagttcgattcgtccacaattaaaaatatctcttctgcaaaaggcctggacgtttgggacagctggccattacaaaacactgacggcactgtcgcaaactatcacggctaccacatcgtctttgcattagccggagatcctaaaaatgcggatgacacatcgatttacatgttctatcaaaaagtcggcgaaacttctattgacagctggaaaaacgctggccgcgtctttaaagacagcgacaaattcgatgcaaatgattctatcctaaaagaccaaacacaagaatggtcaggttcagccacatttacatctgacggaaaaatccgtttattctacactgatttctccggtaaacattacggcaaacaaacactgacaactgcacaagttaacgtatcagcatcagacagctctttgaacatcaacggtgtagaggattataaatcaatctttgacggtgacggaaaaacgtatcaaaatgtacagcagttcatcgatgaaggcaactacagctcaggcgacaaccatacgctgagagatcctcactacgtagaagataaaggccacaaatacttagtatttgaagcaaacactggaactgaagatggctaccaaggcgaagaatctttatttaacaaagcatactatggcaaaagcacatcattcttccgtcaagaaagtcaaaaacttctgcaaagcgataaaaaacgcacggctgagttagcaaacggcgctctcggtatgattgagctaaacgatgattacacactgaaaaaagtgatgaaaccgctgattgcatctaacacagtaacagatgaaattgaacgcgcgaacgtctttaaaatgaacggcaaatggtacctgttcactgactcccgcggatcaaaaatgacgattgacggcattacgtctaacgatatttacatgcttggttatgtttctaattctttaactggcccatacaagccgctgaacaaaactggccttgtgttaaaaatggatcttgatcctaacgatgtaacctttacttactcacacttcgctgtacctcaagcgaaaggaaacaatgtcgtgattacaagctatatgacaaacagaggattctacgcagacaaacaatcaacgtttgcgcctagcttcctgctgaacatcaaaggcaagaaaacatctgttgtcaaagacagcatccttgaacaaggacaattaacagttaacaaataaaaacgcaaaagaaaatgccgatatcctattggcattggaagacata

SEQ ID NO: 10 - DNA, 3877 bp, Artificial Sequence
  pVTSEIII Vector
gcgatgcgtctcgactcctcgacgtcaggtggcacttttcggggaaatgtgcgcggaacccctatttgtttatttttctaaatacattcaaatatgtatccgctcatgagacaataaccctgataaatgcttcaataatattgaaaaaggaagagtatgagtattcaacatttccgtgtcgcccttattcccttttttgcggcattttgccttcctgtttttgctcacccagaaacgctggtgaaagtaaaagatgctgaagatcagttgggtgcacgagtgggttacatcgaactggatctcaacagcggtaagatccttgagagttttcgccccgaagaacgttttccaatgatgagcacttttaaagttctgctatgtggcgcggtattatcccgtattgacgccgggcaagagcaactcggtcgccgcatacactattctcagaatgacttggttgagtactcaccagtcacagaaaagcatcttacggatggcatgacagtaagagaattatgcagtgctgccataaccatgagtgataacactgcggccaacttacttctgacaacgatcggaggaccgaaggagctaaccgcttttttgcacaacatgggggatcatgtaactcgccttgatcgttgggaaccggagctgaatgaagccataccaaacgacgagcgtgacaccacgatgcctgtagcaatggcaacaacgttgcgcaaactattaactggcgaactacttactctagcttcccggcaacaattaatagactggatggaggcggataaagttgcaggaccacttctgcgctcggcccttccggctggctggtttattgctgataaatctggagccggtgagcgtggttctcgcggtatcattgcagcactggggccagatggtaagccctcccgtatcgtagttatctacacgacggggagtcaggcaactatggatgaacgaaatagacagatcgctgagataggtgcctcactgattaagcattggtaactgtcagaccaagtttactcatatatactttagattgatttaaaacttcatttttaatttaaaaggatctaggtgaagatcctttttgataatctcatgaccaaaatcccttaacgtgagttttcgttccactgagcgtcagaccccgtagaaaagatcaaaggatcttcttgagatcctttttttctgcgcgtaatctgctgcttgcaaacaaaaaaaccaccgctaccagcggtggtttgtttgccggatcaagagctaccaactctttttccgaaggtaactggcttcagcagagcgcagataccaaatactgttcttctagtgtagccgtagttaggccaccacttcaagaactctgtagcaccgcctacatacctcgctctgctaatcctgttaccagtggctgctgccagtggcgataagtcgtgtcttaccgggttggactcaagacgatagttaccggataaggcgcagcggtcgggctgaacggggggttcgtgcacacagcccagcttggagcgaacgacctacaccgaactgagatacctacagcgtgagctatgagaaagcgccacgcttcccgaagggagaaaggcggacaggtatccggtaagcggcagggtcggaacaggagagcgcacgagggagcttccagggggaaacgcctggtatctttatagtcctgtcgggtttcgccacctctgacttgagcgtcgatttttgtgatgctcgtcaggggggcggagcctatggaaaaacgccagcaacgcggcctttttacggttcctggccttttgctggccttttgctcacatgttctttcctgcgttatcccctgattctgtggataaccgtattaccgcctttgagtggaggagtcgagacgcatcgctagatgaagagcaggttagatagtcttcgacgtccacatatacgtgccgttcactattatttagtgaaatgagatattatgatattttctgaattgtgattaaaaaggcaactttatgcccatgcaacagaaactataaaaaatacagagaatgaaaagaaacagatagattttttagttctttaggcccgtagtctgcaaatccttttatgattttctatcaaacaaaagaggaaaatagaccagttgcaatccaaacgagagtctaatagaatgaggtcgaaaagtaaatcgcgcgggtttgttactgataaagcaggcaagacctaaaatgtgtaaagggcaaagtgtatactttggcgtcaccccttacatattttaggtctttttttattgtgcgtaactaacttgccatcttcaaacaggagggctggaagaagcagaccgctaacacagtacataaaaaaggagacatgaacgatgaacatcaaaaagtttgcaaaacaagcaacagtattaacctttactaccgcactgctggcaggaggcgcaactcaagcgtttgcgaaagaaacgaaccaaaagccatataaggaaacatacggcatttcccatattacacgccatgatatgctgcaaatccctgaacagcaaaaaaatgaaaaatataaagttcctgagttcgattcgtccacaattaaaaatatctcttctgcaaaaggcctggacgtttgggacagctggccattacaaaacactgacggcactgtcgcaaactatcacggctaccacatcgtctttgcattagccggagatcctaaaaatgcggatgacacatcgatttacatgttctatcaaaaagtcggcgaaacttctattgacagctggaaaaacgctggccgcgtctttaaagacagcgacaaattcgatgcaaatgattctatcctaaaagaccaaacacaagaatggtcaggttcagccacatttacatctgacggaaaaatccgtttattctacactgatttctccggtaaacattacggcaaacaaacactgacaactgcacaagttaacgtatcagcatcagacagctctttgaacatcaacggtgtagaggattataaatcaatctttgacggtgacggaaaaacgtatcaaaatgtacagcagttcatcgatgaaggcaactacagctcaggcgacaaccatacgctgagagatcctcactacgtagaagataaaggccacaaatacttagtatttgaagcaaacactggaactgaagatggctaccaaggcgaagaatctttatttaacaaagcatactatggcaaaagcacatcattcttccgtcaagaaagtcaaaaacttctgcaaagcgataaaaaacgcacggctgagttagcaaacggcgctctcggtatgattgagctaaacgatgattacacactgaaaaaagtgatgaaaccgctgattgcatctaacacagtaacagatgaaattgaacgcgcgaacgtctttaaaatgaacggcaaatggtacctgttcactgactcccgcggatcaaaaatgacgattgacggcattacgtctaacgatatttacatgcttggttatgtttctaattctttaactggcccatacaagccgctgaacaaaactggccttgtgttaaaaatggatcttgatcctaacgatgtaacctttacttactcacacttcgctgtacctcaagcgaaaggaaacaatgtcgtgattacaagctatatgacaaacagaggattctacgcagacaaacaatcaacgtttgcgcctagcttcctgctgaacatcaaaggcaagaaaacatctgttgtcaaagacagcatccttgaacaaggacaattaacagttaacaaataaaaacgcaaaagaaaatgccgatatcctattggcattggaagacataagcacctgctcttctaa

SEQ ID NO: 11 - DNA, 5415 bp, Artificial Sequence
  pYVTSD Vector
ccaaagacgaaaggttgaatgaaacctttttgccatccgacatccacaggtccattctcacacataagtgccaaacgcaacaggaggggatacactagcagcagaccgttgcaaacgcaggacctccactcctcttctcctcaacacccacttttgccatcgaaaaaccagcccagttattgggcttgattggagctcgctcattccaattccttctattaggctactaacaccatgactttattagcctgtctatcctggcccccctggcgaggttcatgtttgtttatttccgaatgcaacaagctccgcattacacccgaacatcactccagatgagggctttctgagtgtggggtcaaatagtttcatgttccccaaatggcccaaaactgacagtttaaacgctgtcttggaacctaatatgacaaaagcgtgatctcatccaagatgaactaagtttggttcgttgaaatgctaacggccagttggtcaaaaagaaacttccaaaagtcggcataccgtttgtcttgtttggtattgattgacgaatgctcaaaaataatctcattaatgcttagcgcagtctctctatcgcttctgaaccccggtgcacctgtgccgaaacgcaaatggggaaacacccgctttttggatgattatgcattgtctccacattgtatgcttccaagattctggtgggaatactgctgatagcctaacgttcatgatcaaaatttaactgttctaacccctacttgacagcaatatataaacagaaggaagctgccctgtcttaaacctttttttttatcatcattattagcttactttcataattgcgactggttccaattgacaagcttttgattttaacgacttttaacgacaacttgagaagatcaaaaaacaactaattattcgaaacgatgagatttccttcaatttttactgctgttttattcgcagcatcctccgcattagctgctccagtcaacactacaacagaagatgaaacggcacaaattccggctgaagctgtcatcggttactcagatttagaaggggatttcgatgttgctgttttgccattttccaacagcacaaataacgggttattgtttataaatactactattgccagcattgctgctaaagaagaaggggtatctctcgagaaaagagaggctgaagccatggagaccgacgtccacatatacctgccgttcactattatttagtgaaatgagatattatgatattttctgaattgtgattaaaaaggcaactttatgcccatgcaacagaaactataaaaaatacagagaatgaaaagaaacagatagattttttagttctttaggcccgtagtctgcaaatccttttatgattttctatcaaacaaaagaggaaaatagaccagttgcaatccaaacgagagtctaatagaatgaggtcgaaaagtaaatcgcgcgggtttgttactgataaagcaggcaagacctaaaatgtgtaaagggcaaagtgtatactttggcgtcaccccttacatattttaggtctttttttattgtgcgtaactaacttgccatcttcaaacaggagggctggaagaagcagaccgctaacacagtacataaaaaaggagacatgaacgatgaacatcaaaaagtttgcaaaacaagcaacagtattaacctttactaccgcactgctggcaggaggcgcaactcaagcgtttgcgaaagaaacgaaccaaaagccatataaggaaacatacggcatttcccatattacacgccatgatatgctgcaaatccctgaacagcaaaaaaatgaaaaatataaagttcctgagttcgattcgtccacaattaaaaatatctcttctgcaaaaggcctggacgtttgggacagctggccattacaaaacactgacggcactgtcgcaaactatcacggctaccacatcgtctttgcattagccggagatcctaaaaatgcggatgacacatcgatttacatgttctatcaaaaagtcggcgaaacttctattgacagctggaaaaacgctggccgcgtctttaaagacagcgacaaattcgatgcaaatgattctatcctaaaagaccaaacacaagaatggtcaggttcagccacatttacatctgacggaaaaatccgtttattctacactgatttctccggtaaacattacggcaaacaaacactgacaactgcacaagttaacgtatcagcatcagacagctctttgaacatcaacggtgtagaggattataaatcaatctttgacggtgacggaaaaacgtatcaaaatgtacagcagttcatcgatgaaggcaactacagctcaggcgacaaccatacgctgagagatcctcactacgtagaagataaaggccacaaatacttagtatttgaagcaaacactggaactgaagatggctaccaaggcgaagaatctttatttaacaaagcatactatggcaaaagcacatcattcttccgtcaagaaagtcaaaaacttctgcaaagcgataaaaaacgcacggctgagttagcaaacggcgctctcggtatgattgagctaaacgatgattacacactgaaaaaagtgatgaaaccgctgattgcatctaacacagtaacagatgaaattgaacgcgcgaacgtctttaaaatgaacggcaaatggtacctgttcactgactcccgcggatcaaaaatgacgattgacggcattacgtctaacgatatttacatgcttggttatgtttctaattctttaactggcccatacaagccgctgaacaaaactggccttgtgttaaaaatggatcttgatcctaacgatgtaacctttacttactcacacttcgctgtacctcaagcgaaaggaaacaatgtcgtgattacaagctatatgacaaacagaggattctacgcagacaaacaatcaacgtttgcgcctagcttcctgctgaacatcaaaggcaagaaaacatctgttgtcaaagacagcatccttgaacaaggacaattaacagttaacaaataaaaacgcaaaagaaaatgccgatatcctattggcattgacggtctcaagtaccatcatcatcatcatcattgagtttgtagccttagacatgactgttcctcagttcaagttgggcacttacgagaagaccggtcttgctagattctaatcaagaggatgtcagaatgccatttgcctgagagatgcaggcttcatttttgatacttttttatttgtaacctatatagtataggattttttttgtcattttgtttcttctcgtacgagcttgctcctgatcagcctatctcgcagctgatgaatatcttgtggtaggggtttgggaaaatcattcgagtttgatgtttttcttggtatttcccactcctcttcagagtacagaagattaagtgagacattcgtttgtgcggatcccccacacaccatagcttcaaaatgtttctactccttttttactcttccagattttctcggactccgcgcatcgccgtaccacttcaaaacacccaagcacagcatactaaattttccctctttcttcctctagggtgtcgttaattacccgtactaaaggtttggaaaagaaaaaagagacagcctcgtttctttttcttcgtcgaaaaaggcaataaaaatttttatcacgtttctttttcttgaaatttttttttttagtttttttctctttcagtgacctccattgatatttaagttaataaacggtcttcaatttctcaagtttcagtttcatttttcttgttctattacaactttttttacttcttgttcattagaaagaaagcatagcaatctaatctaaggggcggtgttgacaattaatcatcggcatagtatatcggcatagtataatacgacaaggtgaggaactaaaccatggccaagttgaccagtgccgttccggtgctcaccgcgcgcgacgtcgccggagcggtcgagttctggaccgaccggctcgggttctcccgggacttcgtggaggacgacttcgccggtgtggtccgggacgacgtgaccctgttcatcagcgcggtccaggaccaggtggtgccggacaacaccctggcctgggtgtgggtgcgcggcctggacgagctgtacgccgagtggtcggaggtcgtgtccacgaacttccgggacgcctccgggccggccatgaccgagatcggcgagcagccgtgggggcgggagttcgccctgcgcgacccggccggcaactgcgtgcacttcgtggccgaggagcaggactgacacgtccgacggcggcccacgggtcccaggcctcggagatccgtcccccttttcctttgtcgatatcatgtaattagttatgtcacgcttacattcacgccctccccccacatccgctctaaccgaaaaggaaggagttagacaacctgaagtctaggtccctatttatttttttatagttatgttagtattaagaacgttatttatatttcaaatttttcttttttttctgtacagacgcgtgtacgcatgtaacattatactgaaaaccttgcttgagaaggttttgggacgctcgaaggctttaatttgcaagctggagactaacatgtgagcaaaaggccagcaaaaggccaggaaccgtaaaaaggccgcgttgctggcgtttttccataggctccgcccccctgacgagcatcacaaaaatcgacgctcaagtcagaggtggcgaaacccgacaggactataaagataccaggcgtttccccctggaagctccctcgtgcgctctcctgttccgaccctgccgcttaccggatacctgtccgcctttctcccttcgggaagcgtggcgctttctcaatgctcacgctgtaggtatctcagttcggtgtaggtcgttcgctccaagctgggctgtgtgcacgaaccccccgttcagcccgaccgctgcgccttatccggtaactatcgtcttgagtccaacccggtaagacacgacttatcgccactggcagcagccactggtaacaggattagcagagcgaggtatgtaggcggtgctacagagttcttgaagtggtggcctaactacggctacactagaaggacagtatttggtatctgcgctctgctgaagccagttaccttcggaaaaagagttggtagctcttgatccggcaaacaaaccaccgctggtagcggtggtttttttgtttgcaagcagcagattacgcgcagaaaaaaaggatctcaagaagatcctttgatcttttctacggggtctgacgctcagtggaacgaaaactcacgttaagggattttggtcatgagatcagatctaacat

SEQ ID NO: 12 - DNA, 3274 bp, Artificial Sequence
  pLVTSD Vector
tagtcttataactatactgacaatagaaacattaacaaatctaaaacagtcttaattctatcttgagaaagtattggtaataatattattgtcgataacgcgagcataataaacggctctgattaaattctgaagtttgttagatacaatgatttcgttcgaaggaactacaaaataaattataaggaggcactcaaaatgagtacaaaagattttaacttggatttggtatctgtttcgaagaaagattcaggtgcatcaccacgcattacaagtatttcgctatgtacacccggttgtaaaacaggagactctgcatggatccatgaagaagaagattatctcagctattttaatgtctacagtgatactttctgctgcagccccgttgtcaggtgtttacgctgccatggagaccgacgtgctagctgctactccggacattgacggtctccagtaagaattcgcatgcgagctcgtcgacagatcttctagactcgagtgcatattttcggcaatcttctcaatgagatgctcttcagcatgttcaatgatgtcgattttttattaaaacgtctcaaaatcgtttctgagacgttttagcgtttatttcgtttagttatcggcataatcgttaaaacaggcgttatcgtagcgtaaaagcccttgagcgtagcgtgctttgcagcgaagatgttgtctgttagattatgaaagccgatgactgaatgaaataataagcgcagcgtccttctatttcggttggaggaggctcaagggagtttgagggaatgaaattccctcatgggtttgattttaaaaattgcttgcaattttgccgagcggtagcgctggaaaatttttgaaaaaaatttggaatttggaaaaaaatggggggaaaggaagcgaattttgcttccgtactacgaccccccattaagtgccgagtgccaatttttgtgccaaaaacgctctatcccaactggctcaagggtttgaggggtttttcaatcgccaacgaatcgccaacgttttcgccaacgttttttataaatctatatttaagtagctttattgttgtttttatgattacaaagtgatacactaattttataaaattatttgattggagttttttaaatggtgatttcagaatcgaaaaaaagagttatgatttctctgacaaaagagcaagataaaaaattaacagatatggcgaaacaaaaaggtttttcaaaatctgcggttgcggcgttagctatagaagaatatgcaagaaaggaatcagaacaaaaaaaataagcgaaagctcgcgtttttagaaggatacgagttttcgctacttgtttttgataaggtaatatatcatggctattaaaaatactaaagctagaaattttggatttttattatatcctgactcaattcctaatgattggaaagaaaaattagagagtttgggcgtatctatggctgtcagtcctttacacgatatggacgaaaaaaaagataaagatacatggaatagtagtgatgttatacgaaatggaaagcactataaaaaaccacactatcacgttatatatattgcacgaaatcctgtaacaatagaaagcgttaggaacaagattaagcgaaaattggggaatagttcagttgctcatgttgagatacttgattatatcaaaggttcatatgaatatttgactcatgaatcaaaggacgctattgctaagaataaacatatatacgacaaaaaagatattttgaacattaatgattttgatattgaccgctatataacacttgatgaaagccaaaaaagagaattgaagaatttacttttagatatagtggatgactataatttggtaaatacaaaagatttaatggcttttattcgccttaggggagcggagtttggaattttaaatacgaatgatgtaaaagatattgtttcaacaaactctagcgcctttagattatggtttgagggcaattatcagtgtggatatagagcaagttatgcaaaggttcttgatgctgaaacgggggaaataaaatgacaaacaaagaaaaagagttatttgctgaaaatgaggaattaaaaaaagaaattaaggacttaaaagagcgtattgaaagatacagagaaatggaagttgaattaagtacaacaatagatttattgagaggagggattattgaataaataaaagcccccctgacgaaagtcgacggcaatagttacccttattatcaagataagaaagaaaaggatttttcgctacgctcaaatcctttaaaaaaacacaaaagaccacattttttaatgtggtctttattcttcaactaaagcacccattagttcaacaaacgaaaattggataaagtgggatatttttaaaatatatatttatgttacagtaatattgacttttaaaaaaggattgattctaatgaagaaagcagacaagtaagcctcctaaattcactttagataaaaatttaggaggcatatcaaatgaactttaataaaattgatttagacaattggaagagaaaagagatatttaatcattatttgaaccaacaaacgacttttagtataaccacagaaattgatattagtgttttataccgaaacataaaacaagaaggatataaattttaccctgcatttattttcttagtgacaagggtgataaactcaaatacagcttttagaactggttacaatagcgacggagagttaggttattgggataagttagagccactttatacaatttttgatggtgtatctaaaacattctctggtatttggactcctgtaaagaatgacttcaaagagttttatgatttatacctttctgatgtagagaaatataatggttcggggaaattgtttcccaaaacacctatacctgaaaatgctttttctctttctattattccatggacttcatttactgggtttaacttaaatatcaataataatagtaattaccttctacccattattacagcaggaaaattcattaataaaggtaattcaatatatttaccgctatctttacaggtacatcattctgtttgtgatggttatcatgcaggattgtttatgaactctattcaggaattgtcagataggcctaatgactggcttttataatatgagataatgccgactgtactttttacagtcggttttctaatgtcactaacctgccccgttagttgaagaaggtttttatattacagctccaagatc

SEQ ID NO: 13 - DNA, 7284 bp, Artificial Sequence
  pVTSD1 Vector
taatacgactcactataggggaattgtgagcggataacaattcccctctagaaataattttgtttaactttaagaaggagatatacatatgcaccatcatcatcatcattcttctggtgtagatctgggtaccgagaacctgtacttccaatccatggagaccgacgtccacatatacctgccgttcactattatttagtgaaatgagatattatgatattttctgaattgtgattaaaaaggcaactttatgcccatgcaacagaaactataaaaaatacagagaatgaaaagaaacagatagattttttagttctttaggcccgtagtctgcaaatccttttatgattttctatcaaacaaaagaggaaaatagaccagttgcaatccaaacgagagtctaatagaatgaggtcgaaaagtaaatcgcgcgggtttgttactgataaagcaggcaagacctaaaatgtgtaaagggcaaagtgtatactttggcgtcaccccttacatattttaggtctttttttattgtgcgtaactaacttgccatcttcaaacaggagggctggaagaagcagaccgctaacacagtacataaaaaaggagacatgaacgatgaacatcaaaaagtttgcaaaacaagcaacagtattaacctttactaccgcactgctggcaggaggcgcaactcaagcgtttgcgaaagaaacgaaccaaaagccatataaggaaacatacggcatttcccatattacacgccatgatatgctgcaaatccctgaacagcaaaaaaatgaaaaatataaagttcctgagttcgattcgtccacaattaaaaatatctcttctgcaaaaggcctggacgtttgggacagctggccattacaaaacactgacggcactgtcgcaaactatcacggctaccacatcgtctttgcattagccggagatcctaaaaatgcggatgacacatcgatttacatgttctatcaaaaagtcggcgaaacttctattgacagctggaaaaacgctggccgcgtctttaaagacagcgacaaattcgatgcaaatgattctatcctaaaagaccaaacacaagaatggtcaggttcagccacatttacatctgacggaaaaatccgtttattctacactgatttctccggtaaacattacggcaaacaaacactgacaactgcacaagttaacgtatcagcatcagacagctctttgaacatcaacggtgtagaggattataaatcaatctttgacggtgacggaaaaacgtatcaaaatgtacagcagttcatcgatgaaggcaactacagctcaggcgacaaccatacgctgagagatcctcactacgtagaagataaaggccacaaatacttagtatttgaagcaaacactggaactgaagatggctaccaaggcgaagaatctttatttaacaaagcatactatggcaaaagcacatcattcttccgtcaagaaagtcaaaaacttctgcaaagcgataaaaaacgcacggctgagttagcaaacggcgctctcggtatgattgagctaaacgatgattacacactgaaaaaagtgatgaaaccgctgattgcatctaacacagtaacagatgaaattgaacgcgcgaacgtctttaaaatgaacggcaaatggtacctgttcactgactcccgcggatcaaaaatgacgattgacggcattacgtctaacgatatttacatgcttggttatgtttctaattctttaactggcccatacaagccgctgaacaaaactggccttgtgttaaaaatggatcttgatcctaacgatgtaacctttacttactcacacttcgctgtacctcaagcgaaaggaaacaatgtcgtgattacaagctatatgacaaacagaggattctacgcagacaaacaatcaacgtttgcgcctagcttcctgctgaacatcaaaggcaagaaaacatctgttgtcaaagacagcatccttgaacaaggacaattaacagttaacaaataaaaacgcaaaagaaaatgccgatatcctattggcattgacggtctccagtaaaggtggatacggatccgaattcgagctccgtcgacaagcttgcggccgcactcgagcaccaccaccaccaccactgagatccggctgctaacaaagcccgaaaggaagctgagttggctgctgccaccgctgagcaataactagcataaccccttggggcctctaaacgggtcttgaggggttttttgctgaaaggaggaactatatccggattggcgaatgggacgcgccctgtagcggcgcattaagcgcggcgggtgtggtggttacgcgcagcgtgaccgctacacttgccagcgccctagcgcccgctcctttcgctttcttcccttcctttctcgccacgttcgccggctttccccgtcaagctctaaatcgggggctccctttagggttccgatttagtgctttacggcacctcgaccccaaaaaacttgattagggtgatggttcacgtagtgggccatcgccctgatagacggtttttcgccctttgacgttggagtccacgttctttaatagtggactcttgttccaaactggaacaacactcaaccctatctcggtctattcttttgatttataagggattttgccgatttcggcctattggttaaaaaatgagctgatttaacaaaaatttaacgcgaattttaacaaaatattaacgtttacaatttcaggtggcacttttcggggaaatgtgcgcggaacccctatttgtttatttttctaaatacattcaaatatgtatccgctcatgaattaattcttagaaaaactcatcgagcatcaaatgaaactgcaatttattcatatcaggattatcaataccatatttttgaaaaagccgtttctgtaatgaaggagaaaactcaccgaggcagttccataggatggcaagatcctggtatcggtctgcgattccgactcgtccaacatcaatacaacctattaatttcccctcgtcaaaaataaggttatcaagtgagaaatcaccatgagtgacgactgaatccggtgagaatggcaaaagtttatgcatttctttccagacttgttcaacaggccagccattacgctcgtcatcaaaatcactcgcatcaaccaaaccgttattcattcgtgattgcgcctgagcgagacgaaatacgcgatcgctgttaaaaggacaattacaaacaggaatcgaatgcaaccggcgcaggaacactgccagcgcatcaacaatattttcacctgaatcaggatattcttctaatacctggaatgctgttttcccggggatcgcagtggtgagtaaccatgcatcatcaggagtacggataaaatgcttgatggtcggaagaggcataaattccgtcagccagtttagtctgaccatctcatctgtaacatcattggcaacgctacctttgccatgtttcagaaacaactctggcgcatcgggcttcccatacaatcgatagattgtcgcacctgattgcccgacattatcgcgagcccatttatacccatataaatcagcatccatgttggaatttaatcgcggcctagagcaagacgtttcccgttgaatatggctcataacaccccttgtattactgtttatgtaagcagacagttttattgttcatgaccaaaatcccttaacgtgagttttcgttccactgagcgtcagaccccgtagaaaagatcaaaggatcttcttgagatcctttttttctgcgcgtaatctgctgcttgcaaacaaaaaaaccaccgctaccagcggtggtttgtttgccggatcaagagctaccaactctttttccgaaggtaactggcttcagcagagcgcagataccaaatactgtccttctagtgtagccgtagttaggccaccacttcaagaactctgtagcaccgcctacatacctcgctctgctaatcctgttaccagtggctgctgccagtggcgataagtcgtgtcttaccgggttggactcaagacgatagttaccggataaggcgcagcggtcgggctgaacggggggttcgtgcacacagcccagcttggagcgaacgacctacaccgaactgagatacctacagcgtgagctatgagaaagcgccacgcttcccgaagggagaaaggcggacaggtatccggtaagcggcagggtcggaacaggagagcgcacgagggagcttccagggggaaacgcctggtatctttatagtcctgtcgggtttcgccacctctgacttgagcgtcgatttttgtgatgctcgtcaggggggcggagcctatggaaaaacgccagcaacgcggcctttttacggttcctggccttttgctggccttttgctcacatgttctttcctgcgttatcccctgattctgtggataaccgtattaccgcctttgagtgagctgataccgctcgccgcagccgaacgaccgagcgcagcgagtcagtgagcgaggaagcggaagagcgcctgatgcggtattttctccttacgcatctgtgcggtatttcacaccgcatatatggtgcactctcagtacaatctgctctgatgccgcatagttaagccagtatacactccgctatcgctacgtgactgggtcatggctgcgccccgacacccgccaacacccgctgacgcgccctgacgggcttgtctgctcccggcatccgcttacagacaagctgtgaccgtctccgggagctgcatgtgtcagaggttttcaccgtcatcaccgaaacgcgcgaggcagctgcggtaaagctcatcagcgtggtcgtgaagcgattcacagatgtctgcctgttcatccgcgtccagctcgttgagtttctccagaagcgttaatgtctggcttctgataaagcgggccatgttaagggcggttttttcctgtttggtcactgatgcctccgtgtaagggggatttctgttcatgggggtaatgataccgatgaaacgagagaggatgctcacgatacgggttactgatgatgaacatgcccggttactggaacgttgtgagggtaaacaactggcggtatggatgcggcgggaccagagaaaaatcactcagggtcaatgccagcgcttcgttaatacagatgtaggtgttccacagggtagccagcagcatcctgcgatgcagatccggaacataatggtgcagggcgctgacttccgcgtttccagactttacgaaacacggaaaccgaagaccattcatgttgttgctcaggtcgcagacgttttgcagcagcagtcgcttcacgttcgctcgcgtatcggtgattcattctgctaaccagtaaggcaaccccgccagcctagccgggtcctcaacgacaggagcacgatcatgcgcacccgtggggccgccatgccggcgataatggcctgcttctcgccgaaacgtttggtggcgggaccagtgacgaaggcttgagcgagggcgtgcaagattccgaataccgcaagcgacaggccgatcatcgtcgcgctccagcgaaagcggtcctcgccgaaaatgacccagagcgctgccggcacctgtcctacgagttgcatgataaagaagacagtcataagtgcggcgacgatagtcatgccccgcgcccaccggaaggagctgactgggttgaaggctctcaagggcatcggtcgagatcccggtgcctaatgagtgagctaacttacattaattgcgttgcgctcactgcccgctttccagtcgggaaacctgtcgtgccagctgcattaatgaatcggccaacgcgcggggagaggcggtttgcgtattgggcgccagggtggtttttcttttcaccagtgagacgggcaacagctgattgcccttcaccgcctggccctgagagagttgcagcaagcggtccacgctggtttgccccagcaggcgaaaatcctgtttgatggtggttaacggcgggatataacatgagctgtcttcggtatcgtcgtatcccactaccgagatatccgcaccaacgcgcagcccggactcggtaatggcgcgcattgcgcccagcgccatctgatcgttggcaaccagcatcgcagtgggaacgatgccctcattcagcatttgcatggtttgttgaaaaccggacatggcactccagtcgccttcccgttccgctatcggctgaatttgattgcgagtgagatatttatgccagccagccagacgcagacgcgccgagacagaacttaatgggcccgctaacagcgcgatttgctggtgacccaatgcgaccagatgctccacgcccagtcgcgtaccgtcttcatgggagaaaataatactgttgatgggtgtctggtcagagacatcaagaaataacgccggaacattagtgcaggcagcttccacagcaatggcatcctggtcatccagcggatagttaatgatcagcccactgacgcgttgcgcgagaagattgtgcaccgccgctttacaggcttcgacgccgcttcgttctaccatcgacaccaccacgctggcacccagttgatcggcgcgagatttaatcgccgcgacaatttgcgacggcgcgtgcagggccagactggaggtggcaacgccaatcagcaacgactgtttgcccgccagttgttgtgccacgcggttgggaatgtaattcagctccgccatcgccgcttccactttttcccgcgttttcgcagaaacgtggctggcctggttcaccacgcgggaaacggtctgataagagacaccggcatactctgcgacatcgtataacgttactggtttcacattcaccaccctgaattgactctcttccgggcgctatcatgccataccgcgaaaggttttgcgccattcgatggtgtccgggatctcgacgctctcccttatgcgactcctgcattaggaagcagcccagtagtaggttgaggccgttgagcaccgccgccgcaaggaatggtgcatgcaaggagatggcgcccaacagtcccccggccacggggcctgccaccatacccacgccgaaacaagcgctcatgagcccgaagtggcgagcccgatcttccccatcggtgatgtcggcgatataggcgccagcaaccgcacctgtggcgccggtgatgccggccacgatgcgtccggcgtagaggatcgagatctcgatcccgcgaaat

SEQ ID NO: 14 - DNA, 7227 bp, Artificial Sequence
  pVTSD2 Vector
taatacgactcactataggggaattgtgagcggataacaattcccctctagaaataattttgtttaactttaagaaggagatataaccatggagaccgacgtccacatatacctgccgttcactattatttagtgaaatgagatattatgatattttctgaattgtgattaaaaaggcaactttatgcccatgcaacagaaactataaaaaatacagagaatgaaaagaaacagatagattttttagttctttaggcccgtagtctgcaaatccttttatgattttctatcaaacaaaagaggaaaatagaccagttgcaatccaaacgagagtctaatagaatgaggtcgaaaagtaaatcgcgcgggtttgttactgataaagcaggcaagacctaaaatgtgtaaagggcaaagtgtatactttggcgtcaccccttacatattttaggtctttttttattgtgcgtaactaacttgccatcttcaaacaggagggctggaagaagcagaccgctaacacagtacataaaaaaggagacatgaacgatgaacatcaaaaagtttgcaaaacaagcaacagtattaacctttactaccgcactgctggcaggaggcgcaactcaagcgtttgcgaaagaaacgaaccaaaagccatataaggaaacatacggcatttcccatattacacgccatgatatgctgcaaatccctgaacagcaaaaaaatgaaaaatataaagttcctgagttcgattcgtccacaattaaaaatatctcttctgcaaaaggcctggacgtttgggacagctggccattacaaaacactgacggcactgtcgcaaactatcacggctaccacatcgtctttgcattagccggagatcctaaaaatgcggatgacacatcgatttacatgttctatcaaaaagtcggcgaaacttctattgacagctggaaaaacgctggccgcgtctttaaagacagcgacaaattcgatgcaaatgattctatcctaaaagaccaaacacaagaatggtcaggttcagccacatttacatctgacggaaaaatccgtttattctacactgatttctccggtaaacattacggcaaacaaacactgacaactgcacaagttaacgtatcagcatcagacagctctttgaacatcaacggtgtagaggattataaatcaatctttgacggtgacggaaaaacgtatcaaaatgtacagcagttcatcgatgaaggcaactacagctcaggcgacaaccatacgctgagagatcctcactacgtagaagataaaggccacaaatacttagtatttgaagcaaacactggaactgaagatggctaccaaggcgaagaatctttatttaacaaagcatactatggcaaaagcacatcattcttccgtcaagaaagtcaaaaacttctgcaaagcgataaaaaacgcacggctgagttagcaaacggcgctctcggtatgattgagctaaacgatgattacacactgaaaaaagtgatgaaaccgctgattgcatctaacacagtaacagatgaaattgaacgcgcgaacgtctttaaaatgaacggcaaatggtacctgttcactgactcccgcggatcaaaaatgacgattgacggcattacgtctaacgatatttacatgcttggttatgtttctaattctttaactggcccatacaagccgctgaacaaaactggccttgtgttaaaaatggatcttgatcctaacgatgtaacctttacttactcacacttcgctgtacctcaagcgaaaggaaacaatgtcgtgattacaagctatatgacaaacagaggattctacgcagacaaacaatcaacgtttgcgcctagcttcctgctgaacatcaaaggcaagaaaacatctgttgtcaaagacagcatccttgaacaaggacaattaacagttaacaaataaaaacgcaaaagaaaatgccgatatcctattggcattgacggtctccagtaaggatcctataggtggatacggatccgaattcgagctccgtcgacaagcttgcggccgcactcgagcaccaccaccaccaccactgagatccggctgctaacaaagcccgaaaggaagctgagttggctgctgccaccgctgagcaataactagcataaccccttggggcctctaaacgggtcttgaggggttttttgctgaaaggaggaactatatccggattggcgaatgggacgcgccctgtagcggcgcattaagcgcggcgggtgtggtggttacgcgcagcgtgaccgctacacttgccagcgccctagcgcccgctcctttcgctttcttcccttcctttctcgccacgttcgccggctttccccgtcaagctctaaatcgggggctccctttagggttccgatttagtgctttacggcacctcgaccccaaaaaacttgattagggtgatggttcacgtagtgggccatcgccctgatagacggtttttcgccctttgacgttggagtccacgttctttaatagtggactcttgttccaaactggaacaacactcaaccctatctcggtctattcttttgatttataagggattttgccgatttcggcctattggttaaaaaatgagctgatttaacaaaaatttaacgcgaattttaacaaaatattaacgtttacaatttcaggtggcacttttcggggaaatgtgcgcggaacccctatttgtttatttttctaaatacattcaaatatgtatccgctcatgaattaattcttagaaaaactcatcgagcatcaaatgaaactgcaatttattcatatcaggattatcaataccatatttttgaaaaagccgtttctgtaatgaaggagaaaactcaccgaggcagttccataggatggcaagatcctggtatcggtctgcgattccgactcgtccaacatcaatacaacctattaatttcccctcgtcaaaaataaggttatcaagtgagaaatcaccatgagtgacgactgaatccggtgagaatggcaaaagtttatgcatttctttccagacttgttcaacaggccagccattacgctcgtcatcaaaatcactcgcatcaaccaaaccgttattcattcgtgattgcgcctgagcgagacgaaatacgcgatcgctgttaaaaggacaattacaaacaggaatcgaatgcaaccggcgcaggaacactgccagcgcatcaacaatattttcacctgaatcaggatattcttctaatacctggaatgctgttttcccggggatcgcagtggtgagtaaccatgcatcatcaggagtacggataaaatgcttgatggtcggaagaggcataaattccgtcagccagtttagtctgaccatctcatctgtaacatcattggcaacgctacctttgccatgtttcagaaacaactctggcgcatcgggcttcccatacaatcgatagattgtcgcacctgattgcccgacattatcgcgagcccatttatacccatataaatcagcatccatgttggaatttaatcgcggcctagagcaagacgtttcccgttgaatatggctcataacaccccttgtattactgtttatgtaagcagacagttttattgttcatgaccaaaatcccttaacgtgagttttcgttccactgagcgtcagaccccgtagaaaagatcaaaggatcttcttgagatcctttttttctgcgcgtaatctgctgcttgcaaacaaaaaaaccaccgctaccagcggtggtttgtttgccggatcaagagctaccaactctttttccgaaggtaactggcttcagcagagcgcagataccaaatactgtccttctagtgtagccgtagttaggccaccacttcaagaactctgtagcaccgcctacatacctcgctctgctaatcctgttaccagtggctgctgccagtggcgataagtcgtgtcttaccgggttggactcaagacgatagttaccggataaggcgcagcggtcgggctgaacggggggttcgtgcacacagcccagcttggagcgaacgacctacaccgaactgagatacctacagcgtgagctatgagaaagcgccacgcttcccgaagggagaaaggcggacaggtatccggtaagcggcagggtcggaacaggagagcgcacgagggagcttccagggggaaacgcctggtatctttatagtcctgtcgggtttcgccacctctgacttgagcgtcgatttttgtgatgctcgtcaggggggcggagcctatggaaaaacgccagcaacgcggcctttttacggttcctggccttttgctggccttttgctcacatgttctttcctgcgttatcccctgattctgtggataaccgtattaccgcctttgagtgagctgataccgctcgccgcagccgaacgaccgagcgcagcgagtcagtgagcgaggaagcggaagagcgcctgatgcggtattttctccttacgcatctgtgcggtatttcacaccgcatatatggtgcactctcagtacaatctgctctgatgccgcatagttaagccagtatacactccgctatcgctacgtgactgggtcatggctgcgccccgacacccgccaacacccgctgacgcgccctgacgggcttgtctgctcccggcatccgcttacagacaagctgtgaccgtctccgggagctgcatgtgtcagaggttttcaccgtcatcaccgaaacgcgcgaggcagctgcggtaaagctcatcagcgtggtcgtgaagcgattcacagatgtctgcctgttcatccgcgtccagctcgttgagtttctccagaagcgttaatgtctggcttctgataaagcgggccatgttaagggcggttttttcctgtttggtcactgatgcctccgtgtaagggggatttctgttcatgggggtaatgataccgatgaaacgagagaggatgctcacgatacgggttactgatgatgaacatgcccggttactggaacgttgtgagggtaaacaactggcggtatggatgcggcgggaccagagaaaaatcactcagggtcaatgccagcgcttcgttaatacagatgtaggtgttccacagggtagccagcagcatcctgcgatgcagatccggaacataatggtgcagggcgctgacttccgcgtttccagactttacgaaacacggaaaccgaagaccattcatgttgttgctcaggtcgcagacgttttgcagcagcagtcgcttcacgttcgctcgcgtatcggtgattcattctgctaaccagtaaggcaaccccgccagcctagccgggtcctcaacgacaggagcacgatcatgcgcacccgtggggccgccatgccggcgataatggcctgcttctcgccgaaacgtttggtggcgggaccagtgacgaaggcttgagcgagggcgtgcaagattccgaataccgcaagcgacaggccgatcatcgtcgcgctccagcgaaagcggtcctcgccgaaaatgacccagagcgctgccggcacctgtcctacgagttgcatgataaagaagacagtcataagtgcggcgacgatagtcatgccccgcgcccaccggaaggagctgactgggttgaaggctctcaagggcatcggtcgagatcccggtgcctaatgagtgagctaacttacattaattgcgttgcgctcactgcccgctttccagtcgggaaacctgtcgtgccagctgcattaatgaatcggccaacgcgcggggagaggcggtttgcgtattgggcgccagggtggtttttcttttcaccagtgagacgggcaacagctgattgcccttcaccgcctggccctgagagagttgcagcaagcggtccacgctggtttgccccagcaggcgaaaatcctgtttgatggtggttaacggcgggatataacatgagctgtcttcggtatcgtcgtatcccactaccgagatatccgcaccaacgcgcagcccggactcggtaatggcgcgcattgcgcccagcgccatctgatcgttggcaaccagcatcgcagtgggaacgatgccctcattcagcatttgcatggtttgttgaaaaccggacatggcactccagtcgccttcccgttccgctatcggctgaatttgattgcgagtgagatatttatgccagccagccagacgcagacgcgccgagacagaacttaatgggcccgctaacagcgcgatttgctggtgacccaatgcgaccagatgctccacgcccagtcgcgtaccgtcttcatgggagaaaataatactgttgatgggtgtctggtcagagacatcaagaaataacgccggaacattagtgcaggcagcttccacagcaatggcatcctggtcatccagcggatagttaatgatcagcccactgacgcgttgcgcgagaagattgtgcaccgccgctttacaggcttcgacgccgcttcgttctaccatcgacaccaccacgctggcacccagttgatcggcgcgagatttaatcgccgcgacaatttgcgacggcgcgtgcagggccagactggaggtggcaacgccaatcagcaacgactgtttgcccgccagttgttgtgccacgcggttgggaatgtaattcagctccgccatcgccgcttccactttttcccgcgttttcgcagaaacgtggctggcctggttcaccacgcgggaaacggtctgataagagacaccggcatactctgcgacatcgtataacgttactggtttcacattcaccaccctgaattgactctcttccgggcgctatcatgccataccgcgaaaggttttgcgccattcgatggtgtccgggatctcgacgctctcccttatgcgactcctgcattaggaagcagcccagtagtaggttgaggccgttgagcaccgccgccgcaaggaatggtgcatgcaaggagatggcgcccaacagtcccccggccacggggcctgccaccatacccacgccgaaacaagcgctcatgagcccgaagtggcgagcccgatcttccccatcggtgatgtcggcgatataggcgccagcaaccgcacctgtggcgccggtgatgccggccacgatgcgtccggcgtagaggatcgagatctcgatcccgcgaaat

SEQ ID NO: 15 - DNA, 7202 bp, Artificial Sequence
  pVTSD3 Vector
taatacgactcactataggggaattgtgagcggataacaattcccctctagaaataattttgtttaactttaagaaggagatataaccatggagaccgacgtccacatatacctgccgttcactattatttagtgaaatgagatattatgatattttctgaattgtgattaaaaaggcaactttatgcccatgcaacagaaactataaaaaatacagagaatgaaaagaaacagatagattttttagttctttaggcccgtagtctgcaaatccttttatgattttctatcaaacaaaagaggaaaatagaccagttgcaatccaaacgagagtctaatagaatgaggtcgaaaagtaaatcgcgcgggtttgttactgataaagcaggcaagacctaaaatgtgtaaagggcaaagtgtatactttggcgtcaccccttacatattttaggtctttttttattgtgcgtaactaacttgccatcttcaaacaggagggctggaagaagcagaccgctaacacagtacataaaaaaggagacatgaacgatgaacatcaaaaagtttgcaaaacaagcaacagtattaacctttactaccgcactgctggcaggaggcgcaactcaagcgtttgcgaaagaaacgaaccaaaagccatataaggaaacatacggcatttcccatattacacgccatgatatgctgcaaatccctgaacagcaaaaaaatgaaaaatataaagttcctgagttcgattcgtccacaattaaaaatatctcttctgcaaaaggcctggacgtttgggacagctggccattacaaaacactgacggcactgtcgcaaactatcacggctaccacatcgtctttgcattagccggagatcctaaaaatgcggatgacacatcgatttacatgttctatcaaaaagtcggcgaaacttctattgacagctggaaaaacgctggccgcgtctttaaagacagcgacaaattcgatgcaaatgattctatcctaaaagaccaaacacaagaatggtcaggttcagccacatttacatctgacggaaaaatccgtttattctacactgatttctccggtaaacattacggcaaacaaacactgacaactgcacaagttaacgtatcagcatcagacagctctttgaacatcaacggtgtagaggattataaatcaatctttgacggtgacggaaaaacgtatcaaaatgtacagcagttcatcgatgaaggcaactacagctcaggcgacaaccatacgctgagagatcctcactacgtagaagataaaggccacaaatacttagtatttgaagcaaacactggaactgaagatggctaccaaggcgaagaatctttatttaacaaagcatactatggcaaaagcacatcattcttccgtcaagaaagtcaaaaacttctgcaaagcgataaaaaacgcacggctgagttagcaaacggcgctctcggtatgattgagctaaacgatgattacacactgaaaaaagtgatgaaaccgctgattgcatctaacacagtaacagatgaaattgaacgcgcgaacgtctttaaaatgaacggcaaatggtacctgttcactgactcccgcggatcaaaaatgacgattgacggcattacgtctaacgatatttacatgcttggttatgtttctaattctttaactggcccatacaagccgctgaacaaaactggccttgtgttaaaaatggatcttgatcctaacgatgtaacctttacttactcacacttcgctgtacctcaagcgaaaggaaacaatgtcgtgattacaagctatatgacaaacagaggattctacgcagacaaacaatcaacgtttgcgcctagcttcctgctgaacatcaaaggcaagaaaacatctgttgtcaaagacagcatccttgaacaaggacaattaacagttaacaaataaaaacgcaaaagaaaatgccgatatcctattggcattgacggtctccagtaccaccatcatcatcatcattaagtcagcggccgcactcgagcaccaccaccaccaccactgagatccggctgctaacaaagcccgaaaggaagctgagttggctgctgccaccgctgagcaataactagcataaccccttggggcctctaaacgggtcttgaggggttttttgctgaaaggaggaactatatccggattggcgaatgggacgcgccctgtagcggcgcattaagcgcggcgggtgtggtggttacgcgcagcgtgaccgctacacttgccagcgccctagcgcccgctcctttcgctttcttcccttcctttctcgccacgttcgccggctttccccgtcaagctctaaatcgggggctccctttagggttccgatttagtgctttacggcacctcgaccccaaaaaacttgattagggtgatggttcacgtagtgggccatcgccctgatagacggtttttcgccctttgacgttggagtccacgttctttaatagtggactcttgttccaaactggaacaacactcaaccctatctcggtctattcttttgatttataagggattttgccgatttcggcctattggttaaaaaatgagctgatttaacaaaaatttaacgcgaattttaacaaaatattaacgtttacaatttcaggtggcacttttcggggaaatgtgcgcggaacccctatttgtttatttttctaaatacattcaaatatgtatccgctcatgaattaattcttagaaaaactcatcgagcatcaaatgaaactgcaatttattcatatcaggattatcaataccatatttttgaaaaagccgtttctgtaatgaaggagaaaactcaccgaggcagttccataggatggcaagatcctggtatcggtctgcgattccgactcgtccaacatcaatacaacctattaatttcccctcgtcaaaaataaggttatcaagtgagaaatcaccatgagtgacgactgaatccggtgagaatggcaaaagtttatgcatttctttccagacttgttcaacaggccagccattacgctcgtcatcaaaatcactcgcatcaaccaaaccgttattcattcgtgattgcgcctgagcgagacgaaatacgcgatcgctgttaaaaggacaattacaaacaggaatcgaatgcaaccggcgcaggaacactgccagcgcatcaacaatattttcacctgaatcaggatattcttctaatacctggaatgctgttttcccggggatcgcagtggtgagtaaccatgcatcatcaggagtacggataaaatgcttgatggtcggaagaggcataaattccgtcagccagtttagtctgaccatctcatctgtaacatcattggcaacgctacctttgccatgtttcagaaacaactctggcgcatcgggcttcccatacaatcgatagattgtcgcacctgattgcccgacattatcgcgagcccatttatacccatataaatcagcatccatgttggaatttaatcgcggcctagagcaagacgtttcccgttgaatatggctcataacaccccttgtattactgtttatgtaagcagacagttttattgttcatgaccaaaatcccttaacgtgagttttcgttccactgagcgtcagaccccgtagaaaagatcaaaggatcttcttgagatcctttttttctgcgcgtaatctgctgcttgcaaacaaaaaaaccaccgctaccagcggtggtttgtttgccggatcaagagctaccaactctttttccgaaggtaactggcttcagcagagcgcagataccaaatactgtccttctagtgtagccgtagttaggccaccacttcaagaactctgtagcaccgcctacatacctcgctctgctaatcctgttaccagtggctgctgccagtggcgataagtcgtgtcttaccgggttggactcaagacgatagttaccggataaggcgcagcggtcgggctgaacggggggttcgtgcacacagcccagcttggagcgaacgacctacaccgaactgagatacctacagcgtgagctatgagaaagcgccacgcttcccgaagggagaaaggcggacaggtatccggtaagcggcagggtcggaacaggagagcgcacgagggagcttccagggggaaacgcctggtatctttatagtcctgtcgggtttcgccacctctgacttgagcgtcgatttttgtgatgctcgtcaggggggcggagcctatggaaaaacgccagcaacgcggcctttttacggttcctggccttttgctggccttttgctcacatgttctttcctgcgttatcccctgattctgtggataaccgtattaccgcctttgagtgagctgataccgctcgccgcagccgaacgaccgagcgcagcgagtcagtgagcgaggaagcggaagagcgcctgatgcggtattttctccttacgcatctgtgcggtatttcacaccgcatatatggtgcactctcagtacaatctgctctgatgccgcatagttaagccagtatacactccgctatcgctacgtgactgggtcatggctgcgccccgacacccgccaacacccgctgacgcgccctgacgggcttgtctgctcccggcatccgcttacagacaagctgtgaccgtctccgggagctgcatgtgtcagaggttttcaccgtcatcaccgaaacgcgcgaggcagctgcggtaaagctcatcagcgtggtcgtgaagcgattcacagatgtctgcctgttcatccgcgtccagctcgttgagtttctccagaagcgttaatgtctggcttctgataaagcgggccatgttaagggcggttttttcctgtttggtcactgatgcctccgtgtaagggggatttctgttcatgggggtaatgataccgatgaaacgagagaggatgctcacgatacgggttactgatgatgaacatgcccggttactggaacgttgtgagggtaaacaactggcggtatggatgcggcgggaccagagaaaaatcactcagggtcaatgccagcgcttcgttaatacagatgtaggtgttccacagggtagccagcagcatcctgcgatgcagatccggaacataatggtgcagggcgctgacttccgcgtttccagactttacgaaacacggaaaccgaagaccattcatgttgttgctcaggtcgcagacgttttgcagcagcagtcgcttcacgttcgctcgcgtatcggtgattcattctgctaaccagtaaggcaaccccgccagcctagccgggtcctcaacgacaggagcacgatcatgcgcacccgtggggccgccatgccggcgataatggcctgcttctcgccgaaacgtttggtggcgggaccagtgacgaaggcttgagcgagggcgtgcaagattccgaataccgcaagcgacaggccgatcatcgtcgcgctccagcgaaagcggtcctcgccgaaaatgacccagagcgctgccggcacctgtcctacgagttgcatgataaagaagacagtcataagtgcggcgacgatagtcatgccccgcgcccaccggaaggagctgactgggttgaaggctctcaagggcatcggtcgagatcccggtgcctaatgagtgagctaacttacattaattgcgttgcgctcactgcccgctttccagtcgggaaacctgtcgtgccagctgcattaatgaatcggccaacgcgcggggagaggcggtttgcgtattgggcgccagggtggtttttcttttcaccagtgagacgggcaacagctgattgcccttcaccgcctggccctgagagagttgcagcaagcggtccacgctggtttgccccagcaggcgaaaatcctgtttgatggtggttaacggcgggatataacatgagctgtcttcggtatcgtcgtatcccactaccgagatatccgcaccaacgcgcagcccggactcggtaatggcgcgcattgcgcccagcgccatctgatcgttggcaaccagcatcgcagtgggaacgatgccctcattcagcatttgcatggtttgttgaaaaccggacatggcactccagtcgccttcccgttccgctatcggctgaatttgattgcgagtgagatatttatgccagccagccagacgcagacgcgccgagacagaacttaatgggcccgctaacagcgcgatttgctggtgacccaatgcgaccagatgctccacgcccagtcgcgtaccgtcttcatgggagaaaataatactgttgatgggtgtctggtcagagacatcaagaaataacgccggaacattagtgcaggcagcttccacagcaatggcatcctggtcatccagcggatagttaatgatcagcccactgacgcgttgcgcgagaagattgtgcaccgccgctttacaggcttcgacgccgcttcgttctaccatcgacaccaccacgctggcacccagttgatcggcgcgagatttaatcgccgcgacaatttgcgacggcgcgtgcagggccagactggaggtggcaacgccaatcagcaacgactgtttgcccgccagttgttgtgccacgcggttgggaatgtaattcagctccgccatcgccgcttccactttttcccgcgttttcgcagaaacgtggctggcctggttcaccacgcgggaaacggtctgataagagacaccggcatactctgcgacatcgtataacgttactggtttcacattcaccaccctgaattgactctcttccgggcgctatcatgccataccgcgaaaggttttgcgccattcgatggtgtccgggatctcgacgctctcccttatgcgactcctgcattaggaagcagcccagtagtaggttgaggccgttgagcaccgccgccgcaaggaatggtgcatgcaaggagatggcgcccaacagtcccccggccacggggcctgccaccatacccacgccgaaacaagcgctcatgagcccgaagtggcgagcccgatcttccccatcggtgatgtcggcgatataggcgccagcaaccgcacctgtggcgccggtgatgccggccacgatgcgtccggcgtagaggatcgagatctcgatcccgcgaaat

SEQ ID NO: 16 - DNA, 5075 bp, Artificial Sequence
  pVTSD4 Vector
cgagggcaaaccatggctcaccatcatcatcatcattcttctggtgtagatctgggtaccgagaacctgtacttccaatccatggagaccgacgtccacatatacctgccgttcactattatttagtgaaatgagatattatgatattttctgaattgtgattaaaaaggcaactttatgcccatgcaacagaaactataaaaaatacagagaatgaaaagaaacagatagattttttagttctttaggcccgtagtctgcaaatccttttatgattttctatcaaacaaaagaggaaaatagaccagttgcaatccaaacgagagtctaatagaatgaggtcgaaaagtaaatcgcgcgggtttgttactgataaagcaggcaagacctaaaatgtgtaaagggcaaagtgtatactttggcgtcaccccttacatattttaggtctttttttattgtgcgtaactaacttgccatcttcaaacaggagggctggaagaagcagaccgctaacacagtacataaaaaaggagacatgaacgatgaacatcaaaaagtttgcaaaacaagcaacagtattaacctttactaccgcactgctggcaggaggcgcaactcaagcgtttgcgaaagaaacgaaccaaaagccatataaggaaacatacggcatttcccatattacacgccatgatatgctgcaaatccctgaacagcaaaaaaatgaaaaatataaagttcctgagttcgattcgtccacaattaaaaatatctcttctgcaaaaggcctggacgtttgggacagctggccattacaaaacactgacggcactgtcgcaaactatcacggctaccacatcgtctttgcattagccggagatcctaaaaatgcggatgacacatcgatttacatgttctatcaaaaagtcggcgaaacttctattgacagctggaaaaacgctggccgcgtctttaaagacagcgacaaattcgatgcaaatgattctatcctaaaagaccaaacacaagaatggtcaggttcagccacatttacatctgacggaaaaatccgtttattctacactgatttctccggtaaacattacggcaaacaaacactgacaactgcacaagttaacgtatcagcatcagacagctctttgaacatcaacggtgtagaggattataaatcaatctttgacggtgacggaaaaacgtatcaaaatgtacagcagttcatcgatgaaggcaactacagctcaggcgacaaccatacgctgagagatcctcactacgtagaagataaaggccacaaatacttagtatttgaagcaaacactggaactgaagatggctaccaaggcgaagaatctttatttaacaaagcatactatggcaaaagcacatcattcttccgtcaagaaagtcaaaaacttctgcaaagcgataaaaaacgcacggctgagttagcaaacggcgctctcggtatgattgagctaaacgatgattacacactgaaaaaagtgatgaaaccgctgattgcatctaacacagtaacagatgaaattgaacgcgcgaacgtctttaaaatgaacggcaaatggtacctgttcactgactcccgcggatcaaaaatgacgattgacggcattacgtctaacgatatttacatgcttggttatgtttctaattctttaactggcccatacaagccgctgaacaaaactggccttgtgttaaaaatggatcttgatcctaacgatgtaacctttacttactcacacttcgctgtacctcaagcgaaaggaaacaatgtcgtgattacaagctatatgacaaacagaggattctacgcagacaaacaatcaacgtttgcgcctagcttcctgctgaacatcaaaggcaagaaaacatctgttgtcaaagacagcatccttgaacaaggacaattaacagttaacaaataaaaacgcaaaagaaaatgccgatatcctattggcattgacggtctcaagtaataaggatccgacctgtgaagtgaaaaatggcgcacattgtgcgacattttttttgtctgccgtttaccgctactgcgtcacggatctccacgcgccctgtagcggcgcattaagcgcggcgggtgtggtggttacgcgcagcgtgaccgctacacttgccagcgccctagcgcccgctcctttcgctttcttcccttcctttctcgccacgttcgccggctttccccgtcaagctctaaatcgggggctccctttagggttccgatttagtgctttacggcacctcgaccccaaaaaacttgattagggtgatggttcacgtagtgggccatcgccctgatagacggtttttcgccctttgacgttggagtccacgttctttaatagtggactcttgttccaaactggaacaacactcaaccctatctcggtctattcttttgatttataagggattttgccgatttcggcctattggttaaaaaatgagctgatttaacaaaaatttaacgcgaattttaacaaaatattaacgcttacaatttcaggtggcacttttcggggaaatgtgcgcggaacccctatttgtttatttttctaaatacattcaaatatgtatccgctcatgagacaataaccctgataaatgcttcaataatattgaaaaaggaagagtatgagccatattcaacgggaaacgtcttgctctaggccgcgattaaattccaacatggatgctgatttatatgggtataaatgggctcgcgataatgtcgggcaatcaggtgcgacaatctatcgattgtatgggaagcccgatgcgccagagttgtttctgaaacatggcaaaggtagcgttgccaatgatgttacagatgagatggtcagactaaactggctgacggaatttatgcctcttccgaccatcaagcattttatccgtactcctgatgatgcatggttactcaccactgcgatccccgggaaaacagcattccaggtattagaagaatatcctgattcaggtgaaaatattgttgatgcgctggcagtgttcctgcgccggttgcattcgattcctgtttgtaattgtccttttaacagcgatcgcgtatttcgtctcgctcaggcgcaatcacgaatgaataacggtttggttgatgcgagtgattttgatgacgagcgtaatggctggcctgttgaacaagtctggaaagaaatgcataaacttttgccattctcaccggattcagtcgtcactcatggtgatttctcacttgataaccttatttttgacgaggggaaattaataggttgtattgatgttggacgagtcggaatcgcagaccgataccaggatcttgccatcctatggaactgcctcggtgagttttctccttcattacagaaacggctttttcaaaaatatggtattgataatcctgatatgaataaattgcagtttcatttgatgctcgatgagtttttctaagaattaatgatgtctcgtttagataaaagtaaagtgattaacagcgcattagagctgcttaatgaggtcggaatcgaaggtttaacaacccgtaaactcgcccagaagctaggtgtagagcagcctacattgtattggcatgtaaaaaataagcgggctttgctcgacgccttagccattgagatgttagataggcaccatactcacttttgccctttagaaggggaaagctggcaagattttttacgtaataacgctaaaagttttagatgtgctttactaagtcatcgcgatggagcaaaagtacatttaggtacacggcctacagaaaaacagtatgaaactctcgaaaatcaattagcctttttatgccaacaaggtttttcactagagaatgcattatatgcactcagcgcagtggggcattttactttaggttgcgtattggaagatcaagagcatcaagtcgctaaagaagaaagggaaacacctactactgatagtatgccgccattattacgacaagctatcgaattatttgatcaccaaggtgcagagccagccttcttattcggccttgaattgatcatatgcggattagaaaaacaacttaaatgtgaaagtgggtcttaaaagcagcataacctttttccgtgatggtaacttcactagtttaaaaggatctaggtgaagatcctttttgataatctcatgaccaaaatcccttaacgtgagttttcgttccactgagcgtcagaccccgtagaaaagatcaaaggatcttcttgagatcctttttttctgcgcgtaatctgctgcttgcaaacaaaaaaaccaccgctaccagcggtggtttgtttgccggatcaagagctaccaactctttttccgaaggtaactggcttcagcagagcgcagataccaaatactgtccttctagtgtagccgtagttaggccaccacttcaagaactctgtagcaccgcctacatacctcgctctgctaatcctgttaccagtggctgctgccagtggcgataagtcgtgtcttaccgggttggactcaagacgatagttaccggataaggcgcagcggtcgggctgaacggggggttcgtgcacacagcccagcttggagcgaacgacctacaccgaactgagatacctacagcgtgagctatgagaaagcgccacgcttcccgaagggagaaaggcggacaggtatccggtaagcggcagggtcggaacaggagagcgcacgagggagcttccagggggaaacgcctggtatctttatagtcctgtcgggtttcgccacctctgacttgagcgtcgatttttgtgatgctcgtcaggggggcggagcctatggaaaaacgccagcaacgcggcctttttacggttcctggccttttgctggccttttgctcacatgacccgacaccatcgaatggccagatgattaattcctaatttttgttgacactctatcattgatagagttattttaccactccctatcagtgatagagaaaagtgaaatgaatagttcgacaaaaatctagataa

SEQ ID NO: 17 - DNA, 7208 bp, Artificial Sequence
  pVTSD5 Vector
taatacgactcactataggggaattgtgagcggataacaattcccctctagaaataattttgtttaactttaagaaggagatatatccatggagaccgacgtccacatatacctgccgttcactattatttagtgaaatgagatattatgatattttctgaattgtgattaaaaaggcaactttatgcccatgcaacagaaactataaaaaatacagagaatgaaaagaaacagatagattttttagttctttaggcccgtagtctgcaaatccttttatgattttctatcaaacaaaagaggaaaatagaccagttgcaatccaaacgagagtctaatagaatgaggtcgaaaagtaaatcgcgcgggtttgttactgataaagcaggcaagacctaaaatgtgtaaagggcaaagtgtatactttggcgtcaccccttacatattttaggtctttttttattgtgcgtaactaacttgccatcttcaaacaggagggctggaagaagcagaccgctaacacagtacataaaaaaggagacatgaacgatgaacatcaaaaagtttgcaaaacaagcaacagtattaacctttactaccgcactgctggcaggaggcgcaactcaagcgtttgcgaaagaaacgaaccaaaagccatataaggaaacatacggcatttcccatattacacgccatgatatgctgcaaatccctgaacagcaaaaaaatgaaaaatataaagttcctgagttcgattcgtccacaattaaaaatatctcttctgcaaaaggcctggacgtttgggacagctggccattacaaaacactgacggcactgtcgcaaactatcacggctaccacatcgtctttgcattagccggagatcctaaaaatgcggatgacacatcgatttacatgttctatcaaaaagtcggcgaaacttctattgacagctggaaaaacgctggccgcgtctttaaagacagcgacaaattcgatgcaaatgattctatcctaaaagaccaaacacaagaatggtcaggttcagccacatttacatctgacggaaaaatccgtttattctacactgatttctccggtaaacattacggcaaacaaacactgacaactgcacaagttaacgtatcagcatcagacagctctttgaacatcaacggtgtagaggattataaatcaatctttgacggtgacggaaaaacgtatcaaaatgtacagcagttcatcgatgaaggcaactacagctcaggcgacaaccatacgctgagagatcctcactacgtagaagataaaggccacaaatacttagtatttgaagcaaacactggaactgaagatggctaccaaggcgaagaatctttatttaacaaagcatactatggcaaaagcacatcattcttccgtcaagaaagtcaaaaacttctgcaaagcgataaaaaacgcacggctgagttagcaaacggcgctctcggtatgattgagctaaacgatgattacacactgaaaaaagtgatgaaaccgctgattgcatctaacacagtaacagatgaaattgaacgcgcgaacgtctttaaaatgaacggcaaatggtacctgttcactgactcccgcggatcaaaaatgacgattgacggcattacgtctaacgatatttacatgcttggttatgtttctaattctttaactggcccatacaagccgctgaacaaaactggccttgtgttaaaaatggatcttgatcctaacgatgtaacctttacttactcacacttcgctgtacctcaagcgaaaggaaacaatgtcgtgattacaagctatatgacaaacagaggattctacgcagacaaacaatcaacgtttgcgcctagcttcctgctgaacatcaaaggcaagaaaacatctgttgtcaaagacagcatccttgaacaaggacaattaacagttaacaaataaaaacgcaaaagaaaatgccgatatcctattggcattgacggtctccagtactggagccacccgcagttcgaaaaataagtcagcggccgcactcgagcaccaccaccaccaccactgagatccggctgctaacaaagcccgaaaggaagctgagttggctgctgccaccgctgagcaataactagcataaccccttggggcctctaaacgggtcttgaggggttttttgctgaaaggaggaactatatccggattggcgaatgggacgcgccctgtagcggcgcattaagcgcggcgggtgtggtggttacgcgcagcgtgaccgctacacttgccagcgccctagcgcccgctcctttcgctttcttcccttcctttctcgccacgttcgccggctttccccgtcaagctctaaatcgggggctccctttagggttccgatttagtgctttacggcacctcgaccccaaaaaacttgattagggtgatggttcacgtagtgggccatcgccctgatagacggtttttcgccctttgacgttggagtccacgttctttaatagtggactcttgttccaaactggaacaacactcaaccctatctcggtctattcttttgatttataagggattttgccgatttcggcctattggttaaaaaatgagctgatttaacaaaaatttaacgcgaattttaacaaaatattaacgtttacaatttcaggtggcacttttcggggaaatgtgcgcggaacccctatttgtttatttttctaaatacattcaaatatgtatccgctcatgaattaattcttagaaaaactcatcgagcatcaaatgaaactgcaatttattcatatcaggattatcaataccatatttttgaaaaagccgtttctgtaatgaaggagaaaactcaccgaggcagttccataggatggcaagatcctggtatcggtctgcgattccgactcgtccaacatcaatacaacctattaatttcccctcgtcaaaaataaggttatcaagtgagaaatcaccatgagtgacgactgaatccggtgagaatggcaaaagtttatgcatttctttccagacttgttcaacaggccagccattacgctcgtcatcaaaatcactcgcatcaaccaaaccgttattcattcgtgattgcgcctgagcgagacgaaatacgcgatcgctgttaaaaggacaattacaaacaggaatcgaatgcaaccggcgcaggaacactgccagcgcatcaacaatattttcacctgaatcaggatattcttctaatacctggaatgctgttttcccggggatcgcagtggtgagtaaccatgcatcatcaggagtacggataaaatgcttgatggtcggaagaggcataaattccgtcagccagtttagtctgaccatctcatctgtaacatcattggcaacgctacctttgccatgtttcagaaacaactctggcgcatcgggcttcccatacaatcgatagattgtcgcacctgattgcccgacattatcgcgagcccatttatacccatataaatcagcatccatgttggaatttaatcgcggcctagagcaagacgtttcccgttgaatatggctcataacaccccttgtattactgtttatgtaagcagacagttttattgttcatgaccaaaatcccttaacgtgagttttcgttccactgagcgtcagaccccgtagaaaagatcaaaggatcttcttgagatcctttttttctgcgcgtaatctgctgcttgcaaacaaaaaaaccaccgctaccagcggtggtttgtttgccggatcaagagctaccaactctttttccgaaggtaactggcttcagcagagcgcagataccaaatactgtccttctagtgtagccgtagttaggccaccacttcaagaactctgtagcaccgcctacatacctcgctctgctaatcctgttaccagtggctgctgccagtggcgataagtcgtgtcttaccgggttggactcaagacgatagttaccggataaggcgcagcggtcgggctgaacggggggttcgtgcacacagcccagcttggagcgaacgacctacaccgaactgagatacctacagcgtgagctatgagaaagcgccacgcttcccgaagggagaaaggcggacaggtatccggtaagcggcagggtcggaacaggagagcgcacgagggagcttccagggggaaacgcctggtatctttatagtcctgtcgggtttcgccacctctgacttgagcgtcgatttttgtgatgctcgtcaggggggcggagcctatggaaaaacgccagcaacgcggcctttttacggttcctggccttttgctggccttttgctcacatgttctttcctgcgttatcccctgattctgtggataaccgtattaccgcctttgagtgagctgataccgctcgccgcagccgaacgaccgagcgcagcgagtcagtgagcgaggaagcggaagagcgcctgatgcggtattttctccttacgcatctgtgcggtatttcacaccgcatatatggtgcactctcagtacaatctgctctgatgccgcatagttaagccagtatacactccgctatcgctacgtgactgggtcatggctgcgccccgacacccgccaacacccgctgacgcgccctgacgggcttgtctgctcccggcatccgcttacagacaagctgtgaccgtctccgggagctgcatgtgtcagaggttttcaccgtcatcaccgaaacgcgcgaggcagctgcggtaaagctcatcagcgtggtcgtgaagcgattcacagatgtctgcctgttcatccgcgtccagctcgttgagtttctccagaagcgttaatgtctggcttctgataaagcgggccatgttaagggcggttttttcctgtttggtcactgatgcctccgtgtaagggggatttctgttcatgggggtaatgataccgatgaaacgagagaggatgctcacgatacgggttactgatgatgaacatgcccggttactggaacgttgtgagggtaaacaactggcggtatggatgcggcgggaccagagaaaaatcactcagggtcaatgccagcgcttcgttaatacagatgtaggtgttccacagggtagccagcagcatcctgcgatgcagatccggaacataatggtgcagggcgctgacttccgcgtttccagactttacgaaacacggaaaccgaagaccattcatgttgttgctcaggtcgcagacgttttgcagcagcagtcgcttcacgttcgctcgcgtatcggtgattcattctgctaaccagtaaggcaaccccgccagcctagccgggtcctcaacgacaggagcacgatcatgcgcacccgtggggccgccatgccggcgataatggcctgcttctcgccgaaacgtttggtggcgggaccagtgacgaaggcttgagcgagggcgtgcaagattccgaataccgcaagcgacaggccgatcatcgtcgcgctccagcgaaagcggtcctcgccgaaaatgacccagagcgctgccggcacctgtcctacgagttgcatgataaagaagacagtcataagtgcggcgacgatagtcatgccccgcgcccaccggaaggagctgactgggttgaaggctctcaagggcatcggtcgagatcccggtgcctaatgagtgagctaacttacattaattgcgttgcgctcactgcccgctttccagtcgggaaacctgtcgtgccagctgcattaatgaatcggccaacgcgcggggagaggcggtttgcgtattgggcgccagggtggtttttcttttcaccagtgagacgggcaacagctgattgcccttcaccgcctggccctgagagagttgcagcaagcggtccacgctggtttgccccagcaggcgaaaatcctgtttgatggtggttaacggcgggatataacatgagctgtcttcggtatcgtcgtatcccactaccgagatatccgcaccaacgcgcagcccggactcggtaatggcgcgcattgcgcccagcgccatctgatcgttggcaaccagcatcgcagtgggaacgatgccctcattcagcatttgcatggtttgttgaaaaccggacatggcactccagtcgccttcccgttccgctatcggctgaatttgattgcgagtgagatatttatgccagccagccagacgcagacgcgccgagacagaacttaatgggcccgctaacagcgcgatttgctggtgacccaatgcgaccagatgctccacgcccagtcgcgtaccgtcttcatgggagaaaataatactgttgatgggtgtctggtcagagacatcaagaaataacgccggaacattagtgcaggcagcttccacagcaatggcatcctggtcatccagcggatagttaatgatcagcccactgacgcgttgcgcgagaagattgtgcaccgccgctttacaggcttcgacgccgcttcgttctaccatcgacaccaccacgctggcacccagttgatcggcgcgagatttaatcgccgcgacaatttgcgacggcgcgtgcagggccagactggaggtggcaacgccaatcagcaacgactgtttgcccgccagttgttgtgccacgcggttgggaatgtaattcagctccgccatcgccgcttccactttttcccgcgttttcgcagaaacgtggctggcctggttcaccacgcgggaaacggtctgataagagacaccggcatactctgcgacatcgtataacgttactggtttcacattcaccaccctgaattgactctcttccgggcgctatcatgccataccgcgaaaggttttgcgccattcgatggtgtccgggatctcgacgctctcccttatgcgactcctgcattaggaagcagcccagtagtaggttgaggccgttgagcaccgccgccgcaaggaatggtgcatgcaaggagatggcgcccaacagtcccccggccacggggcctgccaccatacccacgccgaaacaagcgctcatgagcccgaagtggcgagcccgatcttccccatcggtgatgtcggcgatataggcgccagcaaccgcacctgtggcgccggtgatgccggccacgatgcgtccggcgtagaggatcgagatctcgatcccgcgaaat

SEQ ID NO: 18 - DNA, 7057 bp, Artificial Sequence
  pVTSD6 Vector
gcgcgaggcagcagatcaattcgcgcgcgaaggcgaagcggcatgcataatgtgcctgtcaaatggacgaagcagggattctgcaaaccctatgctactccgtcaagccgtcaattgtctgattcgttaccaattatgacaacttgacggctacatcattcactttttcttcacaaccggcacggaactcgctcgggctggccccggtgcattttttaaatacccgcgagaaatagagttgatcgtcaaaaccaacattgcgaccgacggtggcgataggcatccgggtggtgctcaaaagcagcttcgcctggctgatacgttggtcctcgcgccagcttaagacgctaatccctaactgctggcggaaaagatgtgacagacgcgacggcgacaagcaaacatgctgtgcgacgctggcgatatcaaaattgctgtctgccaggtgatcgctgatgtactgacaagcctcgcgtacccgattatccatcggtggatggagcgactcgttaatcgcttccatgcgccgcagtaacaattgctcaagcagatttatcgccagcagctccgaatagcgcccttccccttgcccggcgttaatgatttgcccaaacaggtcgctgaaatgcggctggtgcgcttcatccgggcgaaagaaccccgtattggcaaatattgacggccagttaagccattcatgccagtaggcgcgcggacgaaagtaaacccactggtgataccattcgcgagcctccggatgacgaccgtagtgatgaatctctcctggcgggaacagcaaaatatcacccggtcggcaaacaaattctcgtccctgatttttcaccaccccctgaccgcgaatggtgagattgagaatataacctttcattcccagcggtcggtcgataaaaaaatcgagataaccgttggcctcaatcggcgttaaacccgccaccagatgggcattaaacgagtatcccggcagcaggggatcattttgcgcttcagccatacttttcatactcccgccattcagagaagaaaccaattgtccatattgcatcagacattgccgtcactgcgtcttttactggctcttctcgctaaccaaaccggtaaccccgcttattaaaagcattctgtaacaaagcgggaccaaagccatgacaaaaacgcgtaacaaaagtgtctataatcacggcagaaaagtccacattgattatttgcacggcgtcacactttgctatgccatagcatttttatccataagattagcggatcctacctgacgctttttatcgcaactctctactgtttctccatacccgtttttttgggctagaaataattttgtttaactttaagaaggagatatacatacccggatctgataaaattattcatctgactgatgattcttttgatactgatgtacttaaggcagatggtgcaatcctggttgatttctgggcacactggtgcggtccgtgcaaaatgatcgctccgattctggatgaaatcgctgacgaatatcagggcaaactgaccgttgcaaaactgaacatcgatcacaacccgggcactgcgccgaaatatggcatccgtggtatcccgactctgctgctgttcaaaaacggtgaagtggcggcaaccaaagtgggtgcactgtctaaaggtcagttgaaagagttcctcgacgctaacctggccggctctggatccggtgatgacgatgacaaggccatggagaccgacgtccacatatacctgccgttcactattatttagtgaaatgagatattatgatattttctgaattgtgattaaaaaggcaactttatgcccatgcaacagaaactataaaaaatacagagaatgaaaagaaacagatagattttttagttctttaggcccgtagtctgcaaatccttttatgattttctatcaaacaaaagaggaaaatagaccagttgcaatccaaacgagagtctaatagaatgaggtcgaaaagtaaatcgcgcgggtttgttactgataaagcaggcaagacctaaaatgtgtaaagggcaaagtgtatactttggcgtcaccccttacatattttaggtctttttttattgtgcgtaactaacttgccatcttcaaacaggagggctggaagaagcagaccgctaacacagtacataaaaaaggagacatgaacgatgaacatcaaaaagtttgcaaaacaagcaacagtattaacctttactaccgcactgctggcaggaggcgcaactcaagcgtttgcgaaagaaacgaaccaaaagccatataaggaaacatacggcatttcccatattacacgccatgatatgctgcaaatccctgaacagcaaaaaaatgaaaaatataaagttcctgagttcgattcgtccacaattaaaaatatctcttctgcaaaaggcctggacgtttgggacagctggccattacaaaacactgacggcactgtcgcaaactatcacggctaccacatcgtctttgcattagccggagatcctaaaaatgcggatgacacatcgatttacatgttctatcaaaaagtcggcgaaacttctattgacagctggaaaaacgctggccgcgtctttaaagacagcgacaaattcgatgcaaatgattctatcctaaaagaccaaacacaagaatggtcaggttcagccacatttacatctgacggaaaaatccgtttattctacactgatttctccggtaaacattacggcaaacaaacactgacaactgcacaagttaacgtatcagcatcagacagctctttgaacatcaacggtgtagaggattataaatcaatctttgacggtgacggaaaaacgtatcaaaatgtacagcagttcatcgatgaaggcaactacagctcaggcgacaaccatacgctgagagatcctcactacgtagaagataaaggccacaaatacttagtatttgaagcaaacactggaactgaagatggctaccaaggcgaagaatctttatttaacaaagcatactatggcaaaagcacatcattcttccgtcaagaaagtcaaaaacttctgcaaagcgataaaaaacgcacggctgagttagcaaacggcgctctcggtatgattgagctaaacgatgattacacactgaaaaaagtgatgaaaccgctgattgcatctaacacagtaacagatgaaattgaacgcgcgaacgtctttaaaatgaacggcaaatggtacctgttcactgactcccgcggatcaaaaatgacgattgacggcattacgtctaacgatatttacatgcttggttatgtttctaattctttaactggcccatacaagccgctgaacaaaactggccttgtgttaaaaatggatcttgatcctaacgatgtaacctttacttactcacacttcgctgtacctcaagcgaaaggaaacaatgtcgtgattacaagctatatgacaaacagaggattctacgcagacaaacaatcaacgtttgcgcctagcttcctgctgaacatcaaaggcaagaaaacatctgttgtcaaagacagcatccttgaacaaggacaattaacagttaacaaataaaaacgcaaaagaaaatgccgatatcctattggcattgacggtctccagtactggagccacccgcagttcgaaaaataagtcagcggccgcactcgagcaccaccaccaccaccactgagatccggctgctaacaaagcccgaaaggaagctgagttggctgctgccaccgctgagcaataactagcataaccccttggggcctctaaacgggtcttgaggggttttttgctgaaaggaggaactatatccggattggcgaatgggacgcgccctgtagcggcgcattaagcgcggcgggtgtggtggttacgcgcagcgtgaccgctacacttgccagcgccctagcgcccgctcctttcgctttcttcccttcctttctcgccacgttcgccggctttccccgtcaagctctaaatcgggggctccctttagggttccgatttagtgctttacggcacctcgaccccaaaaaacttgattagggtgatggttcacgtagtgggccatcgccctgatagacggtttttcgccctttgacgttggagtccacgttctttaatagtggactcttgttccaaactggaacaacactcaaccctatctcggtctattcttttgatttataagggattttgccgatttcggcctattggttaaaaaatgagctgatttaacaaaaatttaacgcgaattttaacaaaatattaacgtttacaatttcaggtggcacttttcggggaaatgtgcgcggaacccctatttgtttatttttctaaatacattcaaatatgtatccgctcatgaattaattcttagaaaaactcatcgagcatcaaatgaaactgcaatttattcatatcaggattatcaataccatatttttgaaaaagccgtttctgtaatgaaggagaaaactcaccgaggcagttccataggatggcaagatcctggtatcggtctgcgattccgactcgtccaacatcaatacaacctattaatttcccctcgtcaaaaataaggttatcaagtgagaaatcaccatgagtgacgactgaatccggtgagaatggcaaaagtttatgcatttctttccagacttgttcaacaggccagccattacgctcgtcatcaaaatcactcgcatcaaccaaaccgttattcattcgtgattgcgcctgagcgagacgaaatacgcgatcgctgttaaaaggacaattacaaacaggaatcgaatgcaaccggcgcaggaacactgccagcgcatcaacaatattttcacctgaatcaggatattcttctaatacctggaatgctgttttcccggggatcgcagtggtgagtaaccatgcatcatcaggagtacggataaaatgcttgatggtcggaagaggcataaattccgtcagccagtttagtctgaccatctcatctgtaacatcattggcaacgctacctttgccatgtttcagaaacaactctggcgcatcgggcttcccatacaatcgatagattgtcgcacctgattgcccgacattatcgcgagcccatttatacccatataaatcagcatccatgttggaatttaatcgcggcctagagcaagacgtttcccgttgaatatggctcataacaccccttgtattactgtttatgtaagcagacagttttattgttcatgaccaaaatcccttaacgtgagttttcgttccactgagcgtcagaccccgtagaaaagatcaaaggatcttcttgagatcctttttttctgcgcgtaatctgctgcttgcaaacaaaaaaaccaccgctaccagcggtggtttgtttgccggatcaagagctaccaactctttttccgaaggtaactggcttcagcagagcgcagataccaaatactgtccttctagtgtagccgtagttaggccaccacttcaagaactctgtagcaccgcctacatacctcgctctgctaatcctgttaccagtggctgctgccagtggcgataagtcgtgtcttaccgggttggactcaagacgatagttaccggataaggcgcagcggtcgggctgaacggggggttcgtgcacacagcccagcttggagcgaacgacctacaccgaactgagatacctacagcgtgagctatgagaaagcgccacgcttcccgaagggagaaaggcggacaggtatccggtaagcggcagggtcggaacaggagagcgcacgagggagcttccagggggaaacgcctggtatctttatagtcctgtcgggtttcgccacctctgacttgagcgtcgatttttgtgatgctcgtcaggggggcggagcctatggaaaaacgccagcaacgcggcctttttacggttcctggccttttgctggccttttgctcacatgttctttcctgcgttatcccctgattctgtggataaccgtattaccgcctttgagtgagctgataccgctcgccgcagccgaacgaccgagcgcagcgagtcagtgagcgaggaagcggaagagcgcctgatgcggtattttctccttacgcatctgtgcggtatttcacaccgcatatatggtgcactctcagtacaatctgctctgatgccgcatagttaagccagtatacactccgctatcgctacgtgactgggtcatggctgcgccccgacacccgccaacacccgctgacgcgccctgacgggcttgtctgctcccggcatccgcttacagacaagctgtgaccgtctccgggagctgcatgtgtcagaggttttcaccgtcatcaccgaaacgcgcgaggcagctgcggtaaagctcatcagcgtggtcgtgaagcgattcacagatgtctgcctgttcatccgcgtccagctcgttgagtttctccagaagcgttaatgtctggcttctgataaagcgggccatgttaagggcggttttttcctgtttggtcactgatgcctccgtgtaagggggatttctgttcatgggggtaatgataccgatgaaacgagagaggatgctcacgatacgggttactgatgatgaacatgcccggttactggaacgttgtgagggtaaacaactggcggtatggatgcggcgggaccagagaaaaatcactcagggtcaatgccagcgcttcgttaatacagatgtaggtgttccacagggtagccagcagcatcctgcgatgcagatccggaacataatggtgcagggcgctgacttccgcgtttccagactttacgaaacacggaaaccgaagaccattcatgttgttgctcaggtcgcagacgttttgcagcagcagtcgcttcacgttcgctcgcgtatcggtgattcattctgctaaccagtaaggcaaccccgccagcctagccgggtcctcaacgacaggagcacgatcatgcgcacccgtgaaac

SEQ ID NO: 19 - DNA, 6701 bp, Artificial Sequence
  pVTSD7 Vector
gcgcgaggcagcagatcaattcgcgcgcgaaggcgaagcggcatgcataatgtgcctgtcaaatggacgaagcagggattctgcaaaccctatgctactccgtcaagccgtcaattgtctgattcgttaccaattatgacaacttgacggctacatcattcactttttcttcacaaccggcacggaactcgctcgggctggccccggtgcattttttaaatacccgcgagaaatagagttgatcgtcaaaaccaacattgcgaccgacggtggcgataggcatccgggtggtgctcaaaagcagcttcgcctggctgatacgttggtcctcgcgccagcttaagacgctaatccctaactgctggcggaaaagatgtgacagacgcgacggcgacaagcaaacatgctgtgcgacgctggcgatatcaaaattgctgtctgccaggtgatcgctgatgtactgacaagcctcgcgtacccgattatccatcggtggatggagcgactcgttaatcgcttccatgcgccgcagtaacaattgctcaagcagatttatcgccagcagctccgaatagcgcccttccccttgcccggcgttaatgatttgcccaaacaggtcgctgaaatgcggctggtgcgcttcatccgggcgaaagaaccccgtattggcaaatattgacggccagttaagccattcatgccagtaggcgcgcggacgaaagtaaacccactggtgataccattcgcgagcctccggatgacgaccgtagtgatgaatctctcctggcgggaacagcaaaatatcacccggtcggcaaacaaattctcgtccctgatttttcaccaccccctgaccgcgaatggtgagattgagaatataacctttcattcccagcggtcggtcgataaaaaaatcgagataaccgttggcctcaatcggcgttaaacccgccaccagatgggcattaaacgagtatcccggcagcaggggatcattttgcgcttcagccatacttttcatactcccgccattcagagaagaaaccaattgtccatattgcatcagacattgccgtcactgcgtcttttactggctcttctcgctaaccaaaccggtaaccccgcttattaaaagcattctgtaacaaagcgggaccaaagccatgacaaaaacgcgtaacaaaagtgtctataatcacggcagaaaagtccacattgattatttgcacggcgtcacactttgctatgccatagcatttttatccataagattagcggatcctacctgacgctttttatcgcaactctctactgtttctccatacccgtttttttgggctagaaataattttgtttaactttaagaaggagatatacatacccatccatggagaccgacgtccacatatacctgccgttcactattatttagtgaaatgagatattatgatattttctgaattgtgattaaaaaggcaactttatgcccatgcaacagaaactataaaaaatacagagaatgaaaagaaacagatagattttttagttctttaggcccgtagtctgcaaatccttttatgattttctatcaaacaaaagaggaaaatagaccagttgcaatccaaacgagagtctaatagaatgaggtcgaaaagtaaatcgcgcgggtttgttactgataaagcaggcaagacctaaaatgtgtaaagggcaaagtgtatactttggcgtcaccccttacatattttaggtctttttttattgtgcgtaactaacttgccatcttcaaacaggagggctggaagaagcagaccgctaacacagtacataaaaaaggagacatgaacgatgaacatcaaaaagtttgcaaaacaagcaacagtattaacctttactaccgcactgctggcaggaggcgcaactcaagcgtttgcgaaagaaacgaaccaaaagccatataaggaaacatacggcatttcccatattacacgccatgatatgctgcaaatccctgaacagcaaaaaaatgaaaaatataaagttcctgagttcgattcgtccacaattaaaaatatctcttctgcaaaaggcctggacgtttgggacagctggccattacaaaacactgacggcactgtcgcaaactatcacggctaccacatcgtctttgcattagccggagatcctaaaaatgcggatgacacatcgatttacatgttctatcaaaaagtcggcgaaacttctattgacagctggaaaaacgctggccgcgtctttaaagacagcgacaaattcgatgcaaatgattctatcctaaaagaccaaacacaagaatggtcaggttcagccacatttacatctgacggaaaaatccgtttattctacactgatttctccggtaaacattacggcaaacaaacactgacaactgcacaagttaacgtatcagcatcagacagctctttgaacatcaacggtgtagaggattataaatcaatctttgacggtgacggaaaaacgtatcaaaatgtacagcagttcatcgatgaaggcaactacagctcaggcgacaaccatacgctgagagatcctcactacgtagaagataaaggccacaaatacttagtatttgaagcaaacactggaactgaagatggctaccaaggcgaagaatctttatttaacaaagcatactatggcaaaagcacatcattcttccgtcaagaaagtcaaaaacttctgcaaagcgataaaaaacgcacggctgagttagcaaacggcgctctcggtatgattgagctaaacgatgattacacactgaaaaaagtgatgaaaccgctgattgcatctaacacagtaacagatgaaattgaacgcgcgaacgtctttaaaatgaacggcaaatggtacctgttcactgactcccgcggatcaaaaatgacgattgacggcattacgtctaacgatatttacatgcttggttatgtttctaattctttaactggcccatacaagccgctgaacaaaactggccttgtgttaaaaatggatcttgatcctaacgatgtaacctttacttactcacacttcgctgtacctcaagcgaaaggaaacaatgtcgtgattacaagctatatgacaaacagaggattctacgcagacaaacaatcaacgtttgcgcctagcttcctgctgaacatcaaaggcaagaaaacatctgttgtcaaagacagcatccttgaacaaggacaattaacagttaacaaataaaaacgcaaaagaaaatgccgatatcctattggcattgacggtctccagtactggagccacccgcagttcgaaaaataagtcagcggccgcactcgagcaccaccaccaccaccactgagatccggctgctaacaaagcccgaaaggaagctgagttggctgctgccaccgctgagcaataactagcataaccccttggggcctctaaacgggtcttgaggggttttttgctgaaaggaggaactatatccggattggcgaatgggacgcgccctgtagcggcgcattaagcgcggcgggtgtggtggttacgcgcagcgtgaccgctacacttgccagcgccctagcgcccgctcctttcgctttcttcccttcctttctcgccacgttcgccggctttccccgtcaagctctaaatcgggggctccctttagggttccgatttagtgctttacggcacctcgaccccaaaaaacttgattagggtgatggttcacgtagtgggccatcgccctgatagacggtttttcgccctttgacgttggagtccacgttctttaatagtggactcttgttccaaactggaacaacactcaaccctatctcggtctattcttttgatttataagggattttgccgatttcggcctattggttaaaaaatgagctgatttaacaaaaatttaacgcgaattttaacaaaatattaacgtttacaatttcaggtggcacttttcggggaaatgtgcgcggaacccctatttgtttatttttctaaatacattcaaatatgtatccgctcatgaattaattcttagaaaaactcatcgagcatcaaatgaaactgcaatttattcatatcaggattatcaataccatatttttgaaaaagccgtttctgtaatgaaggagaaaactcaccgaggcagttccataggatggcaagatcctggtatcggtctgcgattccgactcgtccaacatcaatacaacctattaatttcccctcgtcaaaaataaggttatcaagtgagaaatcaccatgagtgacgactgaatccggtgagaatggcaaaagtttatgcatttctttccagacttgttcaacaggccagccattacgctcgtcatcaaaatcactcgcatcaaccaaaccgttattcattcgtgattgcgcctgagcgagacgaaatacgcgatcgctgttaaaaggacaattacaaacaggaatcgaatgcaaccggcgcaggaacactgccagcgcatcaacaatattttcacctgaatcaggatattcttctaatacctggaatgctgttttcccggggatcgcagtggtgagtaaccatgcatcatcaggagtacggataaaatgcttgatggtcggaagaggcataaattccgtcagccagtttagtctgaccatctcatctgtaacatcattggcaacgctacctttgccatgtttcagaaacaactctggcgcatcgggcttcccatacaatcgatagattgtcgcacctgattgcccgacattatcgcgagcccatttatacccatataaatcagcatccatgttggaatttaatcgcggcctagagcaagacgtttcccgttgaatatggctcataacaccccttgtattactgtttatgtaagcagacagttttattgttcatgaccaaaatcccttaacgtgagttttcgttccactgagcgtcagaccccgtagaaaagatcaaaggatcttcttgagatcctttttttctgcgcgtaatctgctgcttgcaaacaaaaaaaccaccgctaccagcggtggtttgtttgccggatcaagagctaccaactctttttccgaaggtaactggcttcagcagagcgcagataccaaatactgtccttctagtgtagccgtagttaggccaccacttcaagaactctgtagcaccgcctacatacctcgctctgctaatcctgttaccagtggctgctgccagtggcgataagtcgtgtcttaccgggttggactcaagacgatagttaccggataaggcgcagcggtcgggctgaacggggggttcgtgcacacagcccagcttggagcgaacgacctacaccgaactgagatacctacagcgtgagctatgagaaagcgccacgcttcccgaagggagaaaggcggacaggtatccggtaagcggcagggtcggaacaggagagcgcacgagggagcttccagggggaaacgcctggtatctttatagtcctgtcgggtttcgccacctctgacttgagcgtcgatttttgtgatgctcgtcaggggggcggagcctatggaaaaacgccagcaacgcggcctttttacggttcctggccttttgctggccttttgctcacatgttctttcctgcgttatcccctgattctgtggataaccgtattaccgcctttgagtgagctgataccgctcgccgcagccgaacgaccgagcgcagcgagtcagtgagcgaggaagcggaagagcgcctgatgcggtattttctccttacgcatctgtgcggtatttcacaccgcatatatggtgcactctcagtacaatctgctctgatgccgcatagttaagccagtatacactccgctatcgctacgtgactgggtcatggctgcgccccgacacccgccaacacccgctgacgcgccctgacgggcttgtctgctcccggcatccgcttacagacaagctgtgaccgtctccgggagctgcatgtgtcagaggttttcaccgtcatcaccgaaacgcgcgaggcagctgcggtaaagctcatcagcgtggtcgtgaagcgattcacagatgtctgcctgttcatccgcgtccagctcgttgagtttctccagaagcgttaatgtctggcttctgataaagcgggccatgttaagggcggttttttcctgtttggtcactgatgcctccgtgtaagggggatttctgttcatgggggtaatgataccgatgaaacgagagaggatgctcacgatacgggttactgatgatgaacatgcccggttactggaacgttgtgagggtaaacaactggcggtatggatgcggcgggaccagagaaaaatcactcagggtcaatgccagcgcttcgttaatacagatgtaggtgttccacagggtagccagcagcatcctgcgatgcagatccggaacataatggtgcagggcgctgacttccgcgtttccagactttacgaaacacggaaaccgaagaccattcatgttgttgctcaggtcgcagacgttttgcagcagcagtcgcttcacgttcgctcgcgtatcggtgattcattctgctaaccagtaaggcaaccccgccagcctagccgggtcctcaacgacaggagcacgatcatgcgcacccgtgaaac

SEQ ID NO: 20 - DNA, 7051 bp, Artificial Sequence
  pVTSD8 Vector
gcgcgaggcagcagatcaattcgcgcgcgaaggcgaagcggcatgcataatgtgcctgtcaaatggacgaagcagggattctgcaaaccctatgctactccgtcaagccgtcaattgtctgattcgttaccaattatgacaacttgacggctacatcattcactttttcttcacaaccggcacggaactcgctcgggctggccccggtgcattttttaaatacccgcgagaaatagagttgatcgtcaaaaccaacattgcgaccgacggtggcgataggcatccgggtggtgctcaaaagcagcttcgcctggctgatacgttggtcctcgcgccagcttaagacgctaatccctaactgctggcggaaaagatgtgacagacgcgacggcgacaagcaaacatgctgtgcgacgctggcgatatcaaaattgctgtctgccaggtgatcgctgatgtactgacaagcctcgcgtacccgattatccatcggtggatggagcgactcgttaatcgcttccatgcgccgcagtaacaattgctcaagcagatttatcgccagcagctccgaatagcgcccttccccttgcccggcgttaatgatttgcccaaacaggtcgctgaaatgcggctggtgcgcttcatccgggcgaaagaaccccgtattggcaaatattgacggccagttaagccattcatgccagtaggcgcgcggacgaaagtaaacccactggtgataccattcgcgagcctccggatgacgaccgtagtgatgaatctctcctggcgggaacagcaaaatatcacccggtcggcaaacaaattctcgtccctgatttttcaccaccccctgaccgcgaatggtgagattgagaatataacctttcattcccagcggtcggtcgataaaaaaatcgagataaccgttggcctcaatcggcgttaaacccgccaccagatgggcattaaacgagtatcccggcagcaggggatcattttgcgcttcagccatacttttcatactcccgccattcagagaagaaaccaattgtccatattgcatcagacattgccgtcactgcgtcttttactggctcttctcgctaaccaaaccggtaaccccgcttattaaaagcattctgtaacaaagcgggaccaaagccatgacaaaaacgcgtaacaaaagtgtctataatcacggcagaaaagtccacattgattatttgcacggcgtcacactttgctatgccatagcatttttatccataagattagcggatcctacctgacgctttttatcgcaactctctactgtttctccatacccgtttttttgggctagaaataattttgtttaactttaagaaggagatatacatacccggatctgataaaattattcatctgactgatgattcttttgatactgatgtacttaaggcagatggtgcaatcctggttgatttctgggcacactggtgcggtccgtgcaaaatgatcgctccgattctggatgaaatcgctgacgaatatcagggcaaactgaccgttgcaaaactgaacatcgatcacaacccgggcactgcgccgaaatatggcatccgtggtatcccgactctgctgctgttcaaaaacggtgaagtggcggcaaccaaagtgggtgcactgtctaaaggtcagttgaaagagttcctcgacgctaacctggccggctctggatccggtgatgacgatgacaaggccatggagaccgacgtccacatatacctgccgttcactattatttagtgaaatgagatattatgatattttctgaattgtgattaaaaaggcaactttatgcccatgcaacagaaactataaaaaatacagagaatgaaaagaaacagatagattttttagttctttaggcccgtagtctgcaaatccttttatgattttctatcaaacaaaagaggaaaatagaccagttgcaatccaaacgagagtctaatagaatgaggtcgaaaagtaaatcgcgcgggtttgttactgataaagcaggcaagacctaaaatgtgtaaagggcaaagtgtatactttggcgtcaccccttacatattttaggtctttttttattgtgcgtaactaacttgccatcttcaaacaggagggctggaagaagcagaccgctaacacagtacataaaaaaggagacatgaacgatgaacatcaaaaagtttgcaaaacaagcaacagtattaacctttactaccgcactgctggcaggaggcgcaactcaagcgtttgcgaaagaaacgaaccaaaagccatataaggaaacatacggcatttcccatattacacgccatgatatgctgcaaatccctgaacagcaaaaaaatgaaaaatataaagttcctgagttcgattcgtccacaattaaaaatatctcttctgcaaaaggcctggacgtttgggacagctggccattacaaaacactgacggcactgtcgcaaactatcacggctaccacatcgtctttgcattagccggagatcctaaaaatgcggatgacacatcgatttacatgttctatcaaaaagtcggcgaaacttctattgacagctggaaaaacgctggccgcgtctttaaagacagcgacaaattcgatgcaaatgattctatcctaaaagaccaaacacaagaatggtcaggttcagccacatttacatctgacggaaaaatccgtttattctacactgatttctccggtaaacattacggcaaacaaacactgacaactgcacaagttaacgtatcagcatcagacagctctttgaacatcaacggtgtagaggattataaatcaatctttgacggtgacggaaaaacgtatcaaaatgtacagcagttcatcgatgaaggcaactacagctcaggcgacaaccatacgctgagagatcctcactacgtagaagataaaggccacaaatacttagtatttgaagcaaacactggaactgaagatggctaccaaggcgaagaatctttatttaacaaagcatactatggcaaaagcacatcattcttccgtcaagaaagtcaaaaacttctgcaaagcgataaaaaacgcacggctgagttagcaaacggcgctctcggtatgattgagctaaacgatgattacacactgaaaaaagtgatgaaaccgctgattgcatctaacacagtaacagatgaaattgaacgcgcgaacgtctttaaaatgaacggcaaatggtacctgttcactgactcccgcggatcaaaaatgacgattgacggcattacgtctaacgatatttacatgcttggttatgtttctaattctttaactggcccatacaagccgctgaacaaaactggccttgtgttaaaaatggatcttgatcctaacgatgtaacctttacttactcacacttcgctgtacctcaagcgaaaggaaacaatgtcgtgattacaagctatatgacaaacagaggattctacgcagacaaacaatcaacgtttgcgcctagcttcctgctgaacatcaaaggcaagaaaacatctgttgtcaaagacagcatccttgaacaaggacaattaacagttaacaaataaaaacgcaaaagaaaatgccgatatcctattggcattgacggtctccagtaccaccatcatcatcatcattaagtcagcggccgcactcgagcaccaccaccaccaccactgagatccggctgctaacaaagcccgaaaggaagctgagttggctgctgccaccgctgagcaataactagcataaccccttggggcctctaaacgggtcttgaggggttttttgctgaaaggaggaactatatccggattggcgaatgggacgcgccctgtagcggcgcattaagcgcggcgggtgtggtggttacgcgcagcgtgaccgctacacttgccagcgccctagcgcccgctcctttcgctttcttcccttcctttctcgccacgttcgccggctttccccgtcaagctctaaatcgggggctccctttagggttccgatttagtgctttacggcacctcgaccccaaaaaacttgattagggtgatggttcacgtagtgggccatcgccctgatagacggtttttcgccctttgacgttggagtccacgttctttaatagtggactcttgttccaaactggaacaacactcaaccctatctcggtctattcttttgatttataagggattttgccgatttcggcctattggttaaaaaatgagctgatttaacaaaaatttaacgcgaattttaacaaaatattaacgtttacaatttcaggtggcacttttcggggaaatgtgcgcggaacccctatttgtttatttttctaaatacattcaaatatgtatccgctcatgaattaattcttagaaaaactcatcgagcatcaaatgaaactgcaatttattcatatcaggattatcaataccatatttttgaaaaagccgtttctgtaatgaaggagaaaactcaccgaggcagttccataggatggcaagatcctggtatcggtctgcgattccgactcgtccaacatcaatacaacctattaatttcccctcgtcaaaaataaggttatcaagtgagaaatcaccatgagtgacgactgaatccggtgagaatggcaaaagtttatgcatttctttccagacttgttcaacaggccagccattacgctcgtcatcaaaatcactcgcatcaaccaaaccgttattcattcgtgattgcgcctgagcgagacgaaatacgcgatcgctgttaaaaggacaattacaaacaggaatcgaatgcaaccggcgcaggaacactgccagcgcatcaacaatattttcacctgaatcaggatattcttctaatacctggaatgctgttttcccggggatcgcagtggtgagtaaccatgcatcatcaggagtacggataaaatgcttgatggtcggaagaggcataaattccgtcagccagtttagtctgaccatctcatctgtaacatcattggcaacgctacctttgccatgtttcagaaacaactctggcgcatcgggcttcccatacaatcgatagattgtcgcacctgattgcccgacattatcgcgagcccatttatacccatataaatcagcatccatgttggaatttaatcgcggcctagagcaagacgtttcccgttgaatatggctcataacaccccttgtattactgtttatgtaagcagacagttttattgttcatgaccaaaatcccttaacgtgagttttcgttccactgagcgtcagaccccgtagaaaagatcaaaggatcttcttgagatcctttttttctgcgcgtaatctgctgcttgcaaacaaaaaaaccaccgctaccagcggtggtttgtttgccggatcaagagctaccaactctttttccgaaggtaactggcttcagcagagcgcagataccaaatactgtccttctagtgtagccgtagttaggccaccacttcaagaactctgtagcaccgcctacatacctcgctctgctaatcctgttaccagtggctgctgccagtggcgataagtcgtgtcttaccgggttggactcaagacgatagttaccggataaggcgcagcggtcgggctgaacggggggttcgtgcacacagcccagcttggagcgaacgacctacaccgaactgagatacctacagcgtgagctatgagaaagcgccacgcttcccgaagggagaaaggcggacaggtatccggtaagcggcagggtcggaacaggagagcgcacgagggagcttccagggggaaacgcctggtatctttatagtcctgtcgggtttcgccacctctgacttgagcgtcgatttttgtgatgctcgtcaggggggcggagcctatggaaaaacgccagcaacgcggcctttttacggttcctggccttttgctggccttttgctcacatgttctttcctgcgttatcccctgattctgtggataaccgtattaccgcctttgagtgagctgataccgctcgccgcagccgaacgaccgagcgcagcgagtcagtgagcgaggaagcggaagagcgcctgatgcggtattttctccttacgcatctgtgcggtatttcacaccgcatatatggtgcactctcagtacaatctgctctgatgccgcatagttaagccagtatacactccgctatcgctacgtgactgggtcatggctgcgccccgacacccgccaacacccgctgacgcgccctgacgggcttgtctgctcccggcatccgcttacagacaagctgtgaccgtctccgggagctgcatgtgtcagaggttttcaccgtcatcaccgaaacgcgcgaggcagctgcggtaaagctcatcagcgtggtcgtgaagcgattcacagatgtctgcctgttcatccgcgtccagctcgttgagtttctccagaagcgttaatgtctggcttctgataaagcgggccatgttaagggcggttttttcctgtttggtcactgatgcctccgtgtaagggggatttctgttcatgggggtaatgataccgatgaaacgagagaggatgctcacgatacgggttactgatgatgaacatgcccggttactggaacgttgtgagggtaaacaactggcggtatggatgcggcgggaccagagaaaaatcactcagggtcaatgccagcgcttcgttaatacagatgtaggtgttccacagggtagccagcagcatcctgcgatgcagatccggaacataatggtgcagggcgctgacttccgcgtttccagactttacgaaacacggaaaccgaagaccattcatgttgttgctcaggtcgcagacgttttgcagcagcagtcgcttcacgttcgctcgcgtatcggtgattcattctgctaaccagtaaggcaaccccgccagcctagccgggtcctcaacgacaggagcacgatcatgcgcacccgtgaaac

SEQ ID NO: 21 - DNA, 6695 bp, Artificial Sequence
  pVTSD9 Vector
gcgcgaggcagcagatcaattcgcgcgcgaaggcgaagcggcatgcataatgtgcctgtcaaatggacgaagcagggattctgcaaaccctatgctactccgtcaagccgtcaattgtctgattcgttaccaattatgacaacttgacggctacatcattcactttttcttcacaaccggcacggaactcgctcgggctggccccggtgcattttttaaatacccgcgagaaatagagttgatcgtcaaaaccaacattgcgaccgacggtggcgataggcatccgggtggtgctcaaaagcagcttcgcctggctgatacgttggtcctcgcgccagcttaagacgctaatccctaactgctggcggaaaagatgtgacagacgcgacggcgacaagcaaacatgctgtgcgacgctggcgatatcaaaattgctgtctgccaggtgatcgctgatgtactgacaagcctcgcgtacccgattatccatcggtggatggagcgactcgttaatcgcttccatgcgccgcagtaacaattgctcaagcagatttatcgccagcagctccgaatagcgcccttccccttgcccggcgttaatgatttgcccaaacaggtcgctgaaatgcggctggtgcgcttcatccgggcgaaagaaccccgtattggcaaatattgacggccagttaagccattcatgccagtaggcgcgcggacgaaagtaaacccactggtgataccattcgcgagcctccggatgacgaccgtagtgatgaatctctcctggcgggaacagcaaaatatcacccggtcggcaaacaaattctcgtccctgatttttcaccaccccctgaccgcgaatggtgagattgagaatataacctttcattcccagcggtcggtcgataaaaaaatcgagataaccgttggcctcaatcggcgttaaacccgccaccagatgggcattaaacgagtatcccggcagcaggggatcattttgcgcttcagccatacttttcatactcccgccattcagagaagaaaccaattgtccatattgcatcagacattgccgtcactgcgtcttttactggctcttctcgctaaccaaaccggtaaccccgcttattaaaagcattctgtaacaaagcgggaccaaagccatgacaaaaacgcgtaacaaaagtgtctataatcacggcagaaaagtccacattgattatttgcacggcgtcacactttgctatgccatagcatttttatccataagattagcggatcctacctgacgctttttatcgcaactctctactgtttctccatacccgtttttttgggctagaaataattttgtttaactttaagaaggagatatacatacccatccatggagaccgacgtccacatatacctgccgttcactattatttagtgaaatgagatattatgatattttctgaattgtgattaaaaaggcaactttatgcccatgcaacagaaactataaaaaatacagagaatgaaaagaaacagatagattttttagttctttaggcccgtagtctgcaaatccttttatgattttctatcaaacaaaagaggaaaatagaccagttgcaatccaaacgagagtctaatagaatgaggtcgaaaagtaaatcgcgcgggtttgttactgataaagcaggcaagacctaaaatgtgtaaagggcaaagtgtatactttggcgtcaccccttacatattttaggtctttttttattgtgcgtaactaacttgccatcttcaaacaggagggctggaagaagcagaccgctaacacagtacataaaaaaggagacatgaacgatgaacatcaaaaagtttgcaaaacaagcaacagtattaacctttactaccgcactgctggcaggaggcgcaactcaagcgtttgcgaaagaaacgaaccaaaagccatataaggaaacatacggcatttcccatattacacgccatgatatgctgcaaatccctgaacagcaaaaaaatgaaaaatataaagttcctgagttcgattcgtccacaattaaaaatatctcttctgcaaaaggcctggacgtttgggacagctggccattacaaaacactgacggcactgtcgcaaactatcacggctaccacatcgtctttgcattagccggagatcctaaaaatgcggatgacacatcgatttacatgttctatcaaaaagtcggcgaaacttctattgacagctggaaaaacgctggccgcgtctttaaagacagcgacaaattcgatgcaaatgattctatcctaaaagaccaaacacaagaatggtcaggttcagccacatttacatctgacggaaaaatccgtttattctacactgatttctccggtaaacattacggcaaacaaacactgacaactgcacaagttaacgtatcagcatcagacagctctttgaacatcaacggtgtagaggattataaatcaatctttgacggtgacggaaaaacgtatcaaaatgtacagcagttcatcgatgaaggcaactacagctcaggcgacaaccatacgctgagagatcctcactacgtagaagataaaggccacaaatacttagtatttgaagcaaacactggaactgaagatggctaccaaggcgaagaatctttatttaacaaagcatactatggcaaaagcacatcattcttccgtcaagaaagtcaaaaacttctgcaaagcgataaaaaacgcacggctgagttagcaaacggcgctctcggtatgattgagctaaacgatgattacacactgaaaaaagtgatgaaaccgctgattgcatctaacacagtaacagatgaaattgaacgcgcgaacgtctttaaaatgaacggcaaatggtacctgttcactgactcccgcggatcaaaaatgacgattgacggcattacgtctaacgatatttacatgcttggttatgtttctaattctttaactggcccatacaagccgctgaacaaaactggccttgtgttaaaaatggatcttgatcctaacgatgtaacctttacttactcacacttcgctgtacctcaagcgaaaggaaacaatgtcgtgattacaagctatatgacaaacagaggattctacgcagacaaacaatcaacgtttgcgcctagcttcctgctgaacatcaaaggcaagaaaacatctgttgtcaaagacagcatccttgaacaaggacaattaacagttaacaaataaaaacgcaaaagaaaatgccgatatcctattggcattgacggtctccagtaccaccatcatcatcatcattaagtcagcggccgcactcgagcaccaccaccaccaccactgagatccggctgctaacaaagcccgaaaggaagctgagttggctgctgccaccgctgagcaataactagcataaccccttggggcctctaaacgggtcttgaggggttttttgctgaaaggaggaactatatccggattggcgaatgggacgcgccctgtagcggcgcattaagcgcggcgggtgtggtggttacgcgcagcgtgaccgctacacttgccagcgccctagcgcccgctcctttcgctttcttcccttcctttctcgccacgttcgccggctttccccgtcaagctctaaatcgggggctccctttagggttccgatttagtgctttacggcacctcgaccccaaaaaacttgattagggtgatggttcacgtagtgggccatcgccctgatagacggtttttcgccctttgacgttggagtccacgttctttaatagtggactcttgttccaaactggaacaacactcaaccctatctcggtctattcttttgatttataagggattttgccgatttcggcctattggttaaaaaatgagctgatttaacaaaaatttaacgcgaattttaacaaaatattaacgtttacaatttcaggtggcacttttcggggaaatgtgcgcggaacccctatttgtttatttttctaaatacattcaaatatgtatccgctcatgaattaattcttagaaaaactcatcgagcatcaaatgaaactgcaatttattcatatcaggattatcaataccatatttttgaaaaagccgtttctgtaatgaaggagaaaactcaccgaggcagttccataggatggcaagatcctggtatcggtctgcgattccgactcgtccaacatcaatacaacctattaatttcccctcgtcaaaaataaggttatcaagtgagaaatcaccatgagtgacgactgaatccggtgagaatggcaaaagtttatgcatttctttccagacttgttcaacaggccagccattacgctcgtcatcaaaatcactcgcatcaaccaaaccgttattcattcgtgattgcgcctgagcgagacgaaatacgcgatcgctgttaaaaggacaattacaaacaggaatcgaatgcaaccggcgcaggaacactgccagcgcatcaacaatattttcacctgaatcaggatattcttctaatacctggaatgctgttttcccggggatcgcagtggtgagtaaccatgcatcatcaggagtacggataaaatgcttgatggtcggaagaggcataaattccgtcagccagtttagtctgaccatctcatctgtaacatcattggcaacgctacctttgccatgtttcagaaacaactctggcgcatcgggcttcccatacaatcgatagattgtcgcacctgattgcccgacattatcgcgagcccatttatacccatataaatcagcatccatgttggaatttaatcgcggcctagagcaagacgtttcccgttgaatatggctcataacaccccttgtattactgtttatgtaagcagacagttttattgttcatgaccaaaatcccttaacgtgagttttcgttccactgagcgtcagaccccgtagaaaagatcaaaggatcttcttgagatcctttttttctgcgcgtaatctgctgcttgcaaacaaaaaaaccaccgctaccagcggtggtttgtttgccggatcaagagctaccaactctttttccgaaggtaactggcttcagcagagcgcagataccaaatactgtccttctagtgtagccgtagttaggccaccacttcaagaactctgtagcaccgcctacatacctcgctctgctaatcctgttaccagtggctgctgccagtggcgataagtcgtgtcttaccgggttggactcaagacgatagttaccggataaggcgcagcggtcgggctgaacggggggttcgtgcacacagcccagcttggagcgaacgacctacaccgaactgagatacctacagcgtgagctatgagaaagcgccacgcttcccgaagggagaaaggcggacaggtatccggtaagcggcagggtcggaacaggagagcgcacgagggagcttccagggggaaacgcctggtatctttatagtcctgtcgggtttcgccacctctgacttgagcgtcgatttttgtgatgctcgtcaggggggcggagcctatggaaaaacgccagcaacgcggcctttttacggttcctggccttttgctggccttttgctcacatgttctttcctgcgttatcccctgattctgtggataaccgtattaccgcctttgagtgagctgataccgctcgccgcagccgaacgaccgagcgcagcgagtcagtgagcgaggaagcggaagagcgcctgatgcggtattttctccttacgcatctgtgcggtatttcacaccgcatatatggtgcactctcagtacaatctgctctgatgccgcatagttaagccagtatacactccgctatcgctacgtgactgggtcatggctgcgccccgacacccgccaacacccgctgacgcgccctgacgggcttgtctgctcccggcatccgcttacagacaagctgtgaccgtctccgggagctgcatgtgtcagaggttttcaccgtcatcaccgaaacgcgcgaggcagctgcggtaaagctcatcagcgtggtcgtgaagcgattcacagatgtctgcctgttcatccgcgtccagctcgttgagtttctccagaagcgttaatgtctggcttctgataaagcgggccatgttaagggcggttttttcctgtttggtcactgatgcctccgtgtaagggggatttctgttcatgggggtaatgataccgatgaaacgagagaggatgctcacgatacgggttactgatgatgaacatgcccggttactggaacgttgtgagggtaaacaactggcggtatggatgcggcgggaccagagaaaaatcactcagggtcaatgccagcgcttcgttaatacagatgtaggtgttccacagggtagccagcagcatcctgcgatgcagatccggaacataatggtgcagggcgctgacttccgcgtttccagactttacgaaacacggaaaccgaagaccattcatgttgttgctcaggtcgcagacgttttgcagcagcagtcgcttcacgttcgctcgcgtatcggtgattcattctgctaaccagtaaggcaaccccgccagcctagccgggtcctcaacgacaggagcacgatcatgcgcacccgtgaaac